European Patent Application EP 4 653 469 A1, published November 26, 2025. Title: FUSION PROTEIN OF GE AND GI OF VARICELLA-ZOSTER VIRUS AND USE. Applicant: XIAMEN UNIVERSITY. Application CN. The sequence listing filed with the application follows.

SEQUENCE LISTING (72 sequences)

SEQ ID NO: 1 - DNA, 1545 bp, synthetic construct
  source 1..1545: mol_type = other DNA; note = a nucleotide sequence encoding gE(aa.23-537)
cgtataacgaatccggtcagagcatccgtcttgcgatacgatgattttcacatcgatgaagacaaactggatacaaactccgtatatgagccttactaccattcagatcatgcggagtcttcatgggtaaatcggggagagtcttcgcgaaaagcgtacgatcataactcaccttatatatggccacgtaatgattatgatggatttttagagaacgcacacgaacaccatggggtgtataatcagggccgtggtatcgatagcggggaacggttaatgcaacccacacaaatgtctgcacaggaggatcttggggacgatacgggcatccacgttatccctacgttaaacggcgatgacagacataaaattgtaaatgtggaccaacgtcaatacggtgacgtgtttaaaggagatcttaatccaaaaccccaaggccaaagactcattgaggtgtcagtggaagaaaatcacccgtttactttacgcgcaccgattcagcggatttatggagtccggtacaccgagacttggagctttttgccgtcattaacctgtacgggagacgcagcgcccgccatccagcatatatgtttaaaacatacaacatgctttcaagacgtggtggtggatgtggattgcgcggaaaatactaaagaggatcagttggccgaaatcagttaccgttttcaaggtaagaaggaagcggaccaaccgtggattgttgtaaacacgagcacactgtttgatgaactcgaattagacccccccgagattgaaccgggtgtcttgaaagtacttcggacagaaaaacaatacttgggtgtgtacatttggaacatgcgcggctccgatggtacgtctacctacgccacgtttttggtcacctggaaaggggatgaaaaaacaagaaaccctacgcccgcagtaactcctcaaccaagaggggctgagtttcatatgtggaattaccactcgcatgtattttcagttggtgatacgtttagcttggcaatgcatcttcagtataagatacatgaagcgccatttgatttgctgttagagtggttgtatgtccccatcgatcctacatgtcaaccaatgcggttatattctacgtgtttgtatcatcccaacgcaccccaatgcctctctcatatgaattccggttgtacatttacctcgccacatttagcccagcgtgttgcaagcacagtgtatcaaaattgtgaacatgcagataactacaccgcatattgtctgggaatatctcatatggagcctagctttggtctaatcttacacgacgggggcaccacgttaaagtttgtagatacacccgagagtttgtcgggattatacgtttttgtggtgtattttaacgggcatgttgaagccgtagcatacactgttgtatccacagtagatcattttgtaaacgcaattgaagagcgtggatttccgccaacggccggtcagccaccggcgactactaaacccaaggaaattacccccgtaaaccccggaacgtcaccacttctacga

SEQ ID NO: 2 - DNA, 756 bp, synthetic construct
  source 1..756: mol_type = other DNA; note = a nucleotide sequence encoding gI(aa.21-271)
ttgatcttcaagggcgaccacgtgagcttgcaagttaacagcagtctcacgtctatccttattcccatgcaaaatgataattatacagagataaaaggacagcttgtctttattggagagcaactacctaccgggacaaactatagcggaacactggaactgttatacgcggatacggtggcgttttgtttccggtcagtacaagtaataagatacgacggatgtccccggattagaacgagcgcttttatttcgtgtaggtacaaacattcgtggcattatggtaactcaacggatcggatatcaacagagccggatgctggtgtaatgttgaaaattaccaaaccgggaataaatgatgctggtgtgtatgtacttcttgttcggttagaccatagcagatccaccgatggtttcattcttggtgtaaatgtatatacagcgggctcgcatcacaacattcacggggttatctacacttctccatctctacagaatggatattctacaagagccctttttcaacaagctcgtttgtgtgatttacccgcgacacccaaagggtccggtacctccctgtttcaacatatgcttgatcttcgtgccggtaaatcgttagaggataacccttggttacatgaggacgttgttacgacagaaactaagtccgttgttaaggaggggatagaaaatcacgtatatccaacggatatgtccacgttacccgaaaagtcccttaatgatcctccagaataa

SEQ ID NO: 3 - DNA, 60 bp, synthetic construct
  source 1..60: mol_type = other DNA; note = a nucleotide sequence encoding linker
ggagggggagggtcaggagggggagggtcaggagggggagggtcaggagggggagggtca

SEQ ID NO: 4 - DNA, 2391 bp, synthetic construct
  source 1..2391: mol_type = other DNA; note = a nucleotide sequence encoding gE-gI (HIS tag)
cgtataacgaatccggtcagagcatccgtcttgcgatacgatgattttcacatcgatgaagacaaactggatacaaactccgtatatgagccttactaccattcagatcatgcggagtcttcatgggtaaatcggggagagtcttcgcgaaaagcgtacgatcataactcaccttatatatggccacgtaatgattatgatggatttttagagaacgcacacgaacaccatggggtgtataatcagggccgtggtatcgatagcggggaacggttaatgcaacccacacaaatgtctgcacaggaggatcttggggacgatacgggcatccacgttatccctacgttaaacggcgatgacagacataaaattgtaaatgtggaccaacgtcaatacggtgacgtgtttaaaggagatcttaatccaaaaccccaaggccaaagactcattgaggtgtcagtggaagaaaatcacccgtttactttacgcgcaccgattcagcggatttatggagtccggtacaccgagacttggagctttttgccgtcattaacctgtacgggagacgcagcgcccgccatccagcatatatgtttaaaacatacaacatgctttcaagacgtggtggtggatgtggattgcgcggaaaatactaaagaggatcagttggccgaaatcagttaccgttttcaaggtaagaaggaagcggaccaaccgtggattgttgtaaacacgagcacactgtttgatgaactcgaattagacccccccgagattgaaccgggtgtcttgaaagtacttcggacagaaaaacaatacttgggtgtgtacatttggaacatgcgcggctccgatggtacgtctacctacgccacgtttttggtcacctggaaaggggatgaaaaaacaagaaaccctacgcccgcagtaactcctcaaccaagaggggctgagtttcatatgtggaattaccactcgcatgtattttcagttggtgatacgtttagcttggcaatgcatcttcagtataagatacatgaagcgccatttgatttgctgttagagtggttgtatgtccccatcgatcctacatgtcaaccaatgcggttatattctacgtgtttgtatcatcccaacgcaccccaatgcctctctcatatgaattccggttgtacatttacctcgccacatttagcccagcgtgttgcaagcacagtgtatcaaaattgtgaacatgcagataactacaccgcatattgtctgggaatatctcatatggagcctagctttggtctaatcttacacgacgggggcaccacgttaaagtttgtagatacacccgagagtttgtcgggattatacgtttttgtggtgtattttaacgggcatgttgaagccgtagcatacactgttgtatccacagtagatcattttgtaaacgcaattgaagagcgtggatttccgccaacggccggtcagccaccggcgactactaaacccaaggaaattacccccgtaaaccccggaacgtcaccacttctacgaggagggggagggtcaggagggggagggtcaggagggggagggtcaggagggggagggtcattgatcttcaagggcgaccacgtgagcttgcaagttaacagcagtctcacgtctatccttattcccatgcaaaatgataattatacagagataaaaggacagcttgtctttattggagagcaactacctaccgggacaaactatagcggaacactggaactgttatacgcggatacggtggcgttttgtttccggtcagtacaagtaataagatacgacggatgtccccggattagaacgagcgcttttatttcgtgtaggtacaaacattcgtggcattatggtaactcaacggatcggatatcaacagagccggatgctggtgtaatgttgaaaattaccaaaccgggaataaatgatgctggtgtgtatgtacttcttgttcggttagaccatagcagatccaccgatggtttcattcttggtgtaaatgtatatacagcgggctcgcatcacaacattcacggggttatctacacttctccatctctacagaatggatattctacaagagccctttttcaacaagctcgtttgtgtgatttacccgcgacacccaaagggtccggtacctccctgtttcaacatatgcttgatcttcgtgccggtaaatcgttagaggataacccttggttacatgaggacgttgttacgacagaaactaagtccgttgttaaggaggggatagaaaatcacgtatatccaacggatatgtccacgttacccgaaaagtcccttaatgatcctccagaacatcaccaccatcaccaccaccaccatcactaa

SEQ ID NO: 5 - DNA, 2358 bp, synthetic construct
  source 1..2358: mol_type = other DNA; note = a nucleotide sequence encoding gI-gE
ttgatcttcaagggcgaccacgtgagcttgcaagttaacagcagtctcacgtctatccttattcccatgcaaaatgataattatacagagataaaaggacagcttgtctttattggagagcaactacctaccgggacaaactatagcggaacactggaactgttatacgcggatacggtggcgttttgtttccggtcagtacaagtaataagatacgacggatgtccccggattagaacgagcgcttttatttcgtgtaggtacaaacattcgtggcattatggtaactcaacggatcggatatcaacagagccggatgctggtgtaatgttgaaaattaccaaaccgggaataaatgatgctggtgtgtatgtacttcttgttcggttagaccatagcagatccaccgatggtttcattcttggtgtaaatgtatatacagcgggctcgcatcacaacattcacggggttatctacacttctccatctctacagaatggatattctacaagagccctttttcaacaagctcgtttgtgtgatttacccgcgacacccaaagggtccggtacctccctgtttcaacatatgcttgatcttcgtgccggtaaatcgttagaggataacccttggttacatgaggacgttgttacgacagaaactaagtccgttgttaaggaggggatagaaaatcacgtatatccaacggatatgtccacgttacccgaaaagtcccttaatgatcctccagaaggagggggagggtcaggagggggagggtcaggagggggagggtcaggagggggagggtcacgtataacgaatccggtcagagcatccgtcttgcgatacgatgattttcacatcgatgaagacaaactggatacaaactccgtatatgagccttactaccattcagatcatgcggagtcttcatgggtaaatcggggagagtcttcgcgaaaagcgtacgatcataactcaccttatatatggccacgtaatgattatgatggatttttagagaacgcacacgaacaccatggggtgtataatcagggccgtggtatcgatagcggggaacggttaatgcaacccacacaaatgtctgcacaggaggatcttggggacgatacgggcatccacgttatccctacgttaaacggcgatgacagacataaaattgtaaatgtggaccaacgtcaatacggtgacgtgtttaaaggagatcttaatccaaaaccccaaggccaaagactcattgaggtgtcagtggaagaaaatcacccgtttactttacgcgcaccgattcagcggatttatggagtccggtacaccgagacttggagctttttgccgtcattaacctgtacgggagacgcagcgcccgccatccagcatatatgtttaaaacatacaacatgctttcaagacgtggtggtggatgtggattgcgcggaaaatactaaagaggatcagttggccgaaatcagttaccgttttcaaggtaagaaggaagcggaccaaccgtggattgttgtaaacacgagcacactgtttgatgaactcgaattagacccccccgagattgaaccgggtgtcttgaaagtacttcggacagaaaaacaatacttgggtgtgtacatttggaacatgcgcggctccgatggtacgtctacctacgccacgtttttggtcacctggaaaggggatgaaaaaacaagaaaccctacgcccgcagtaactcctcaaccaagaggggctgagtttcatatgtggaattaccactcgcatgtattttcagttggtgatacgtttagcttggcaatgcatcttcagtataagatacatgaagcgccatttgatttgctgttagagtggttgtatgtccccatcgatcctacatgtcaaccaatgcggttatattctacgtgtttgtatcatcccaacgcaccccaatgcctctctcatatgaattccggttgtacatttacctcgccacatttagcccagcgtgttgcaagcacagtgtatcaaaattgtgaacatgcagataactacaccgcatattgtctgggaatatctcatatggagcctagctttggtctaatcttacacgacgggggcaccacgttaaagtttgtagatacacccgagagtttgtcgggattatacgtttttgtggtgtattttaacgggcatgttgaagccgtagcatacactgttgtatccacagtagatcattttgtaaacgcaattgaagagcgtggatttccgccaacggccggtcagccaccggcgactactaaacccaaggaaattacccccgtaaaccccggaacgtcaccacttctacga

SEQ ID NO: 6 - protein, 786 aa, synthetic construct
  source 1..786: note = gE-gI
RITNPVRASVLRYDDFHIDEDKLDTNSVYEPYYHSDHAESSWVNRGESSRKAYDHNSPYIWPRNDYDGFLENAHEHHGVYNQGRGIDSGERLMQPTQMSAQEDLGDDTGIHVIPTLNGDDRHKIVNVDQRQYGDVFKGDLNPKPQGQRLIEVSVEENHPFTLRAPIQRIYGVRYTETWSFLPSLTCTGDAAPAIQHICLKHTTCFQDVVVDVDCAENTKEDQLAEISYRFQGKKEADQPWIVVNTSTLFDELELDPPEIEPGVLKVLRTEKQYLGVYIWNMRGSDGTSTYATFLVTWKGDEKTRNPTPAVTPQPRGAEFHMWNYHSHVFSVGDTFSLAMHLQYKIHEAPFDLLLEWLYVPIDPTCQPMRLYSTCLYHPNAPQCLSHMNSGCTFTSPHLAQRVASTVYQNCEHADNYTAYCLGISHMEPSFGLILHDGGTTLKFVDTPESLSGLYVFVVYFNGHVEAVAYTVVSTVDHFVNAIEERGFPPTAGQPPATTKPKEITPVNPGTSPLLRGGGGSGGGGSGGGGSGGGGSLIFKGDHVSLQVNSSLTSILIPMQNDNYTEIKGQLVFIGEQLPTGTNYSGTLELLYADTVAFCFRSVQVIRYDGCPRIRTSAFISCRYKHSWHYGNSTDRISTEPDAGVMLKITKPGINDAGVYVLLVRLDHSRSTDGFILGVNVYTAGSHHNIHGVIYTSPSLQNGYSTRALFQQARLCDLPATPKGSGTSLFQHMLDLRAGKSLEDNPWLHEDVVTTETKSVVKEGIENHVYPTDMSTLPEKSLNDPPE

SEQ ID NO: 7 - protein, 786 aa, synthetic construct
  source 1..786: note = gI-gE
LIFKGDHVSLQVNSSLTSILIPMQNDNYTEIKGQLVFIGEQLPTGTNYSGTLELLYADTVAFCFRSVQVIRYDGCPRIRTSAFISCRYKHSWHYGNSTDRISTEPDAGVMLKITKPGINDAGVYVLLVRLDHSRSTDGFILGVNVYTAGSHHNIHGVIYTSPSLQNGYSTRALFQQARLCDLPATPKGSGTSLFQHMLDLRAGKSLEDNPWLHEDVVTTETKSVVKEGIENHVYPTDMSTLPEKSLNDPPEGGGGSGGGGSGGGGSGGGGSRITNPVRASVLRYDDFHIDEDKLDTNSVYEPYYHSDHAESSWVNRGESSRKAYDHNSPYIWPRNDYDGFLENAHEHHGVYNQGRGIDSGERLMQPTQMSAQEDLGDDTGIHVIPTLNGDDRHKIVNVDQRQYGDVFKGDLNPKPQGQRLIEVSVEENHPFTLRAPIQRIYGVRYTETWSFLPSLTCTGDAAPAIQHICLKHTTCFQDVVVDVDCAENTKEDQLAEISYRFQGKKEADQPWIVVNTSTLFDELELDPPEIEPGVLKVLRTEKQYLGVYIWNMRGSDGTSTYATFLVTWKGDEKTRNPTPAVTPQPRGAEFHMWNYHSHVFSVGDTFSLAMHLQYKIHEAPFDLLLEWLYVPIDPTCQPMRLYSTCLYHPNAPQCLSHMNSGCTFTSPHLAQRVASTVYQNCEHADNYTAYCLGISHMEPSFGLILHDGGTTLKFVDTPESLSGLYVFVVYFNGHVEAVAYTVVSTVDHFVNAIEERGFPPTAGQPPATTKPKEITPVNPGTSPLLR

SEQ ID NO: 8 - DNA, 30 bp, synthetic construct
  source 1..30: mol_type = other DNA; note = a nucleotide sequence encoding His tag
catcaccaccatcaccaccaccaccatcac

SEQ ID NO: 9 - protein, 10 aa, synthetic construct
  source 1..10: note = His tag
HHHHHHHHHH

SEQ ID NO: 10 - protein, 796 aa, synthetic construct
  source 1..796: note = gE-gI (HIS tag)
RITNPVRASVLRYDDFHIDEDKLDTNSVYEPYYHSDHAESSWVNRGESSRKAYDHNSPYIWPRNDYDGFLENAHEHHGVYNQGRGIDSGERLMQPTQMSAQEDLGDDTGIHVIPTLNGDDRHKIVNVDQRQYGDVFKGDLNPKPQGQRLIEVSVEENHPFTLRAPIQRIYGVRYTETWSFLPSLTCTGDAAPAIQHICLKHTTCFQDVVVDVDCAENTKEDQLAEISYRFQGKKEADQPWIVVNTSTLFDELELDPPEIEPGVLKVLRTEKQYLGVYIWNMRGSDGTSTYATFLVTWKGDEKTRNPTPAVTPQPRGAEFHMWNYHSHVFSVGDTFSLAMHLQYKIHEAPFDLLLEWLYVPIDPTCQPMRLYSTCLYHPNAPQCLSHMNSGCTFTSPHLAQRVASTVYQNCEHADNYTAYCLGISHMEPSFGLILHDGGTTLKFVDTPESLSGLYVFVVYFNGHVEAVAYTVVSTVDHFVNAIEERGFPPTAGQPPATTKPKEITPVNPGTSPLLRGGGGSGGGGSGGGGSGGGGSLIFKGDHVSLQVNSSLTSILIPMQNDNYTEIKGQLVFIGEQLPTGTNYSGTLELLYADTVAFCFRSVQVIRYDGCPRIRTSAFISCRYKHSWHYGNSTDRISTEPDAGVMLKITKPGINDAGVYVLLVRLDHSRSTDGFILGVNVYTAGSHHNIHGVIYTSPSLQNGYSTRALFQQARLCDLPATPKGSGTSLFQHMLDLRAGKSLEDNPWLHEDVVTTETKSVVKEGIENHVYPTDMSTLPEKSLNDPPEHHHHHHHHHH

SEQ ID NO: 11 - protein, 623 aa, synthetic construct
  source 1..623: note = gE in full-length
MGTVNKPVVGVLMGFGIITGTLRITNPVRASVLRYDDFHIDEDKLDTNSVYEPYYHSDHAESSWVNRGESSRKAYDHNSPYIWPRNDYDGFLENAHEHHGVYNQGRGIDSGERLMQPTQMSAQEDLGDDTGIHVIPTLNGDDRHKIVNVDQRQYGDVFKGDLNPKPQGQRLIEVSVEENHPFTLRAPIQRIYGVRYTETWSFLPSLTCTGDAAPAIQHICLKHTTCFQDVVVDVDCAENTKEDQLAEISYRFQGKKEADQPWIVVNTSTLFDELELDPPEIEPGVLKVLRTEKQYLGVYIWNMRGSDGTSTYATFLVTWKGDEKTRNPTPAVTPQPRGAEFHMWNYHSHVFSVGDTFSLAMHLQYKIHEAPFDLLLEWLYVPIDPTCQPMRLYSTCLYHPNAPQCLSHMNSGCTFTSPHLAQRVASTVYQNCEHADNYTAYCLGISHMEPSFGLILHDGGTTLKFVDTPESLSGLYVFVVYFNGHVEAVAYTVVSTVDHFVNAIEERGFPPTAGQPPATTKPKEITPVNPGTSPLLRYAAWTGGLAAVVLLCLVIFLICTAKRMRVKAYRVDKSPYNQSMYYAGLPVDDFEDSESTDTEEEFGNAIGGSHGGSSYTVYIDKTR

SEQ ID NO: 12 - protein, 354 aa, synthetic construct
  source 1..354: note = gI in full-length
MFLIQCLISAVIFYIQVTNALIFKGDHVSLQVNSSLTSILIPMQNDNYTEIKGQLVFIGEQLPTGTNYSGTLELLYADTVAFCFRSVQVIRYDGCPRIRTSAFISCRYKHSWHYGNSTDRISTEPDAGVMLKITKPGINDAGVYVLLVRLDHSRSTDGFILGVNVYTAGSHHNIHGVIYTSPSLQNGYSTRALFQQARLCDLPATPKGSGTSLFQHMLDLRAGKSLEDNPWLHEDVVTTETKSVVKEGIENHVYPTDMSTLPEKSLNDPPENLLIIIPIVASVMILTAMVIVIVISVKRRRIKKHPIYRPNTKTRRGIQNATPESDVMLEAAIAQLATIREESPPHSVVNPFVK

SEQ ID NO: 13 - protein, 515 aa, synthetic construct
  source 1..515: note = gE(aa. 23-537)
RITNPVRASVLRYDDFHIDEDKLDTNSVYEPYYHSDHAESSWVNRGESSRKAYDHNSPYIWPRNDYDGFLENAHEHHGVYNQGRGIDSGERLMQPTQMSAQEDLGDDTGIHVIPTLNGDDRHKIVNVDQRQYGDVFKGDLNPKPQGQRLIEVSVEENHPFTLRAPIQRIYGVRYTETWSFLPSLTCTGDAAPAIQHICLKHTTCFQDVVVDVDCAENTKEDQLAEISYRFQGKKEADQPWIVVNTSTLFDELELDPPEIEPGVLKVLRTEKQYLGVYIWNMRGSDGTSTYATFLVTWKGDEKTRNPTPAVTPQPRGAEFHMWNYHSHVFSVGDTFSLAMHLQYKIHEAPFDLLLEWLYVPIDPTCQPMRLYSTCLYHPNAPQCLSHMNSGCTFTSPHLAQRVASTVYQNCEHADNYTAYCLGISHMEPSFGLILHDGGTTLKFVDTPESLSGLYVFVVYFNGHVEAVAYTVVSTVDHFVNAIEERGFPPTAGQPPATTKPKEITPVNPGTSPLLR

SEQ ID NO: 14 - protein, 251 aa, synthetic construct
  source 1..251: note = gI(aa. 21-271)
LIFKGDHVSLQVNSSLTSILIPMQNDNYTEIKGQLVFIGEQLPTGTNYSGTLELLYADTVAFCFRSVQVIRYDGCPRIRTSAFISCRYKHSWHYGNSTDRISTEPDAGVMLKITKPGINDAGVYVLLVRLDHSRSTDGFILGVNVYTAGSHHNIHGVIYTSPSLQNGYSTRALFQQARLCDLPATPKGSGTSLFQHMLDLRAGKSLEDNPWLHEDVVTTETKSVVKEGIENHVYPTDMSTLPEKSLNDPPE

SEQ ID NO: 15 - protein, 20 aa, synthetic construct
  source 1..20: note = linker
GGGGSGGGGSGGGGSGGGGS

SEQ ID NO: 16 - DNA, 17 bp, synthetic construct
  source 1..17: mol_type = other DNA; note = T7 promotor
taatacgactcactata

SEQ ID NO: 17 - RNA, 47 nt, synthetic construct
  source 1..47: mol_type = other RNA; note = 5 UTR
agaataaactagtattcttctggtccccacagactcagagagaaccc

SEQ ID NO: 18 - RNA, 295 nt, synthetic construct
  source 1..295: mol_type = other RNA; note = 3 UTR
ctcgagctggtactgcatgcacgcaatgctagctgcccctttcccgtcctgggtaccccgagtctcccccgacctcgggtcccaggtatgctcccacctccacctgccccactcaccacctctgctagttccagacacctcccaagcacgcagcaatgcagctcaaaacgcttagcctagccacacccccacgggaaacagcagtgattaacctttagcaataaacgaaagtttaactaagctatactaaccccagggttggtcaatttcgtgccagccacaccctggagctagc

SEQ ID NO: 19 - RNA, 110 nt, synthetic construct
  source 1..110: mol_type = other RNA; note = polyA
aaaaaaaaaaaaaaaaaaaaaaaaaaaaaagcatatgactaaaaaaaaaaaaaaaaaaaaaaaaaaaaaaaaaaaaaaaaaaaaaaaaaaaaaaaaaaaaaaaaaaaaaa

SEQ ID NO: 20 - protein, 786 aa, synthetic construct
  source 1..786: note = fusion protein gEgI(gE-I40T)
RITNPVRASVLRYDDFHTDEDKLDTNSVYEPYYHSDHAESSWVNRGESSRKAYDHNSPYIWPRNDYDGFLENAHEHHGVYNQGRGIDSGERLMQPTQMSAQEDLGDDTGIHVIPTLNGDDRHKIVNVDQRQYGDVFKGDLNPKPQGQRLIEVSVEENHPFTLRAPIQRIYGVRYTETWSFLPSLTCTGDAAPAIQHICLKHTTCFQDVVVDVDCAENTKEDQLAEISYRFQGKKEADQPWIVVNTSTLFDELELDPPEIEPGVLKVLRTEKQYLGVYIWNMRGSDGTSTYATFLVTWKGDEKTRNPTPAVTPQPRGAEFHMWNYHSHVFSVGDTFSLAMHLQYKIHEAPFDLLLEWLYVPIDPTCQPMRLYSTCLYHPNAPQCLSHMNSGCTFTSPHLAQRVASTVYQNCEHADNYTAYCLGISHMEPSFGLILHDGGTTLKFVDTPESLSGLYVFVVYFNGHVEAVAYTVVSTVDHFVNAIEERGFPPTAGQPPATTKPKEITPVNPGTSPLLRGGGGSGGGGSGGGGSGGGGSLIFKGDHVSLQVNSSLTSILIPMQNDNYTEIKGQLVFIGEQLPTGTNYSGTLELLYADTVAFCFRSVQVIRYDGCPRIRTSAFISCRYKHSWHYGNSTDRISTEPDAGVMLKITKPGINDAGVYVLLVRLDHSRSTDGFILGVNVYTAGSHHNIHGVIYTSPSLQNGYSTRALFQQARLCDLPATPKGSGTSLFQHMLDLRAGKSLEDNPWLHEDVVTTETKSVVKEGIENHVYPTDMSTLPEKSLNDPPE

SEQ ID NO: 21 - protein, 786 aa, synthetic construct
  source 1..786: note = fusion protein gEgI(gE-E124D)
RITNPVRASVLRYDDFHIDEDKLDTNSVYEPYYHSDHAESSWVNRGESSRKAYDHNSPYIWPRNDYDGFLENAHEHHGVYNQGRGIDSGERLMQPTQMSAQDDLGDDTGIHVIPTLNGDDRHKIVNVDQRQYGDVFKGDLNPKPQGQRLIEVSVEENHPFTLRAPIQRIYGVRYTETWSFLPSLTCTGDAAPAIQHICLKHTTCFQDVVVDVDCAENTKEDQLAEISYRFQGKKEADQPWIVVNTSTLFDELELDPPEIEPGVLKVLRTEKQYLGVYIWNMRGSDGTSTYATFLVTWKGDEKTRNPTPAVTPQPRGAEFHMWNYHSHVFSVGDTFSLAMHLQYKIHEAPFDLLLEWLYVPIDPTCQPMRLYSTCLYHPNAPQCLSHMNSGCTFTSPHLAQRVASTVYQNCEHADNYTAYCLGISHMEPSFGLILHDGGTTLKFVDTPESLSGLYVFVVYFNGHVEAVAYTVVSTVDHFVNAIEERGFPPTAGQPPATTKPKEITPVNPGTSPLLRGGGGSGGGGSGGGGSGGGGSLIFKGDHVSLQVNSSLTSILIPMQNDNYTEIKGQLVFIGEQLPTGTNYSGTLELLYADTVAFCFRSVQVIRYDGCPRIRTSAFISCRYKHSWHYGNSTDRISTEPDAGVMLKITKPGINDAGVYVLLVRLDHSRSTDGFILGVNVYTAGSHHNIHGVIYTSPSLQNGYSTRALFQQARLCDLPATPKGSGTSLFQHMLDLRAGKSLEDNPWLHEDVVTTETKSVVKEGIENHVYPTDMSTLPEKSLNDPPE

SEQ ID NO: 22 - protein, 786 aa, synthetic construct
  source 1..786: note = fusion protein gEgI(gE-L162R)
RITNPVRASVLRYDDFHIDEDKLDTNSVYEPYYHSDHAESSWVNRGESSRKAYDHNSPYIWPRNDYDGFLENAHEHHGVYNQGRGIDSGERLMQPTQMSAQEDLGDDTGIHVIPTLNGDDRHKIVNVDQRQYGDVFKGDRNPKPQGQRLIEVSVEENHPFTLRAPIQRIYGVRYTETWSFLPSLTCTGDAAPAIQHICLKHTTCFQDVVVDVDCAENTKEDQLAEISYRFQGKKEADQPWIVVNTSTLFDELELDPPEIEPGVLKVLRTEKQYLGVYIWNMRGSDGTSTYATFLVTWKGDEKTRNPTPAVTPQPRGAEFHMWNYHSHVFSVGDTFSLAMHLQYKIHEAPFDLLLEWLYVPIDPTCQPMRLYSTCLYHPNAPQCLSHMNSGCTFTSPHLAQRVASTVYQNCEHADNYTAYCLGISHMEPSFGLILHDGGTTLKFVDTPESLSGLYVFVVYFNGHVEAVAYTVVSTVDHFVNAIEERGFPPTAGQPPATTKPKEITPVNPGTSPLLRGGGGSGGGGSGGGGSGGGGSLIFKGDHVSLQVNSSLTSILIPMQNDNYTEIKGQLVFIGEQLPTGTNYSGTLELLYADTVAFCFRSVQVIRYDGCPRIRTSAFISCRYKHSWHYGNSTDRISTEPDAGVMLKITKPGINDAGVYVLLVRLDHSRSTDGFILGVNVYTAGSHHNIHGVIYTSPSLQNGYSTRALFQQARLCDLPATPKGSGTSLFQHMLDLRAGKSLEDNPWLHEDVVTTETKSVVKEGIENHVYPTDMSTLPEKSLNDPPE

SEQ ID NO: 23 - protein, 786 aa, synthetic construct
  source 1..786: note = fusion protein gEgI(gE-W319R)
RITNPVRASVLRYDDFHIDEDKLDTNSVYEPYYHSDHAESSWVNRGESSRKAYDHNSPYIWPRNDYDGFLENAHEHHGVYNQGRGIDSGERLMQPTQMSAQEDLGDDTGIHVIPTLNGDDRHKIVNVDQRQYGDVFKGDLNPKPQGQRLIEVSVEENHPFTLRAPIQRIYGVRYTETWSFLPSLTCTGDAAPAIQHICLKHTTCFQDVVVDVDCAENTKEDQLAEISYRFQGKKEADQPWIVVNTSTLFDELELDPPEIEPGVLKVLRTEKQYLGVYIWNMRGSDGTSTYATFLVTRKGDEKTRNPTPAVTPQPRGAEFHMWNYHSHVFSVGDTFSLAMHLQYKIHEAPFDLLLEWLYVPIDPTCQPMRLYSTCLYHPNAPQCLSHMNSGCTFTSPHLAQRVASTVYQNCEHADNYTAYCLGISHMEPSFGLILHDGGTTLKFVDTPESLSGLYVFVVYFNGHVEAVAYTVVSTVDHFVNAIEERGFPPTAGQPPATTKPKEITPVNPGTSPLLRGGGGSGGGGSGGGGSGGGGSLIFKGDHVSLQVNSSLTSILIPMQNDNYTEIKGQLVFIGEQLPTGTNYSGTLELLYADTVAFCFRSVQVIRYDGCPRIRTSAFISCRYKHSWHYGNSTDRISTEPDAGVMLKITKPGINDAGVYVLLVRLDHSRSTDGFILGVNVYTAGSHHNIHGVIYTSPSLQNGYSTRALFQQARLCDLPATPKGSGTSLFQHMLDLRAGKSLEDNPWLHEDVVTTETKSVVKEGIENHVYPTDMSTLPEKSLNDPPE

SEQ ID NO: 24 - protein, 786 aa, synthetic construct
  source 1..786: note = fusion protein gEgI(gE-L359S)
RITNPVRASVLRYDDFHIDEDKLDTNSVYEPYYHSDHAESSWVNRGESSRKAYDHNSPYIWPRNDYDGFLENAHEHHGVYNQGRGIDSGERLMQPTQMSAQEDLGDDTGIHVIPTLNGDDRHKIVNVDQRQYGDVFKGDLNPKPQGQRLIEVSVEENHPFTLRAPIQRIYGVRYTETWSFLPSLTCTGDAAPAIQHICLKHTTCFQDVVVDVDCAENTKEDQLAEISYRFQGKKEADQPWIVVNTSTLFDELELDPPEIEPGVLKVLRTEKQYLGVYIWNMRGSDGTSTYATFLVTWKGDEKTRNPTPAVTPQPRGAEFHMWNYHSHVFSVGDTFSSAMHLQYKIHEAPFDLLLEWLYVPIDPTCQPMRLYSTCLYHPNAPQCLSHMNSGCTFTSPHLAQRVASTVYQNCEHADNYTAYCLGISHMEPSFGLILHDGGTTLKFVDTPESLSGLYVFVVYFNGHVEAVAYTVVSTVDHFVNAIEERGFPPTAGQPPATTKPKEITPVNPGTSPLLRGGGGSGGGGSGGGGSGGGGSLIFKGDHVSLQVNSSLTSILIPMQNDNYTEIKGQLVFIGEQLPTGTNYSGTLELLYADTVAFCFRSVQVIRYDGCPRIRTSAFISCRYKHSWHYGNSTDRISTEPDAGVMLKITKPGINDAGVYVLLVRLDHSRSTDGFILGVNVYTAGSHHNIHGVIYTSPSLQNGYSTRALFQQARLCDLPATPKGSGTSLFQHMLDLRAGKSLEDNPWLHEDVVTTETKSVVKEGIENHVYPTDMSTLPEKSLNDPPE

SEQ ID NO: 25 - protein, 786 aa, synthetic construct
  source 1..786: note = fusion protein gEgI(gE-Q404K)
RITNPVRASVLRYDDFHIDEDKLDTNSVYEPYYHSDHAESSWVNRGESSRKAYDHNSPYIWPRNDYDGFLENAHEHHGVYNQGRGIDSGERLMQPTQMSAQEDLGDDTGIHVIPTLNGDDRHKIVNVDQRQYGDVFKGDLNPKPQGQRLIEVSVEENHPFTLRAPIQRIYGVRYTETWSFLPSLTCTGDAAPAIQHICLKHTTCFQDVVVDVDCAENTKEDQLAEISYRFQGKKEADQPWIVVNTSTLFDELELDPPEIEPGVLKVLRTEKQYLGVYIWNMRGSDGTSTYATFLVTWKGDEKTRNPTPAVTPQPRGAEFHMWNYHSHVFSVGDTFSLAMHLQYKIHEAPFDLLLEWLYVPIDPTCQPMRLYSTCLYHPNAPKCLSHMNSGCTFTSPHLAQRVASTVYQNCEHADNYTAYCLGISHMEPSFGLILHDGGTTLKFVDTPESLSGLYVFVVYFNGHVEAVAYTVVSTVDHFVNAIEERGFPPTAGQPPATTKPKEITPVNPGTSPLLRGGGGSGGGGSGGGGSGGGGSLIFKGDHVSLQVNSSLTSILIPMQNDNYTEIKGQLVFIGEQLPTGTNYSGTLELLYADTVAFCFRSVQVIRYDGCPRIRTSAFISCRYKHSWHYGNSTDRISTEPDAGVMLKITKPGINDAGVYVLLVRLDHSRSTDGFILGVNVYTAGSHHNIHGVIYTSPSLQNGYSTRALFQQARLCDLPATPKGSGTSLFQHMLDLRAGKSLEDNPWLHEDVVTTETKSVVKEGIENHVYPTDMSTLPEKSLNDPPE

SEQ ID NO: 26 - protein, 786 aa, synthetic construct
  source 1..786: note = fusion protein gEgI(gE-L536I)
RITNPVRASVLRYDDFHIDEDKLDTNSVYEPYYHSDHAESSWVNRGESSRKAYDHNSPYIWPRNDYDGFLENAHEHHGVYNQGRGIDSGERLMQPTQMSAQEDLGDDTGIHVIPTLNGDDRHKIVNVDQRQYGDVFKGDLNPKPQGQRLIEVSVEENHPFTLRAPIQRIYGVRYTETWSFLPSLTCTGDAAPAIQHICLKHTTCFQDVVVDVDCAENTKEDQLAEISYRFQGKKEADQPWIVVNTSTLFDELELDPPEIEPGVLKVLRTEKQYLGVYIWNMRGSDGTSTYATFLVTWKGDEKTRNPTPAVTPQPRGAEFHMWNYHSHVFSVGDTFSLAMHLQYKIHEAPFDLLLEWLYVPIDPTCQPMRLYSTCLYHPNAPQCLSHMNSGCTFTSPHLAQRVASTVYQNCEHADNYTAYCLGISHMEPSFGLILHDGGTTLKFVDTPESLSGLYVFVVYFNGHVEAVAYTVVSTVDHFVNAIEERGFPPTAGQPPATTKPKEITPVNPGTSPLIRGGGGSGGGGSGGGGSGGGGSLIFKGDHVSLQVNSSLTSILIPMQNDNYTEIKGQLVFIGEQLPTGTNYSGTLELLYADTVAFCFRSVQVIRYDGCPRIRTSAFISCRYKHSWHYGNSTDRISTEPDAGVMLKITKPGINDAGVYVLLVRLDHSRSTDGFILGVNVYTAGSHHNIHGVIYTSPSLQNGYSTRALFQQARLCDLPATPKGSGTSLFQHMLDLRAGKSLEDNPWLHEDVVTTETKSVVKEGIENHVYPTDMSTLPEKSLNDPPE

SEQ ID NO: 27 - protein, 786 aa, synthetic construct
  source 1..786: note = fusion protein gEgI(gE-I40T, D150N)
RITNPVRASVLRYDDFHTDEDKLDTNSVYEPYYHSDHAESSWVNRGESSRKAYDHNSPYIWPRNDYDGFLENAHEHHGVYNQGRGIDSGERLMQPTQMSAQEDLGDDTGIHVIPTLNGDDRHKIVNVNQRQYGDVFKGDLNPKPQGQRLIEVSVEENHPFTLRAPIQRIYGVRYTETWSFLPSLTCTGDAAPAIQHICLKHTTCFQDVVVDVDCAENTKEDQLAEISYRFQGKKEADQPWIVVNTSTLFDELELDPPEIEPGVLKVLRTEKQYLGVYIWNMRGSDGTSTYATFLVTWKGDEKTRNPTPAVTPQPRGAEFHMWNYHSHVFSVGDTFSLAMHLQYKIHEAPFDLLLEWLYVPIDPTCQPMRLYSTCLYHPNAPQCLSHMNSGCTFTSPHLAQRVASTVYQNCEHADNYTAYCLGISHMEPSFGLILHDGGTTLKFVDTPESLSGLYVFVVYFNGHVEAVAYTVVSTVDHFVNAIEERGFPPTAGQPPATTKPKEITPVNPGTSPLLRGGGGSGGGGSGGGGSGGGGSLIFKGDHVSLQVNSSLTSILIPMQNDNYTEIKGQLVFIGEQLPTGTNYSGTLELLYADTVAFCFRSVQVIRYDGCPRIRTSAFISCRYKHSWHYGNSTDRISTEPDAGVMLKITKPGINDAGVYVLLVRLDHSRSTDGFILGVNVYTAGSHHNIHGVIYTSPSLQNGYSTRALFQQARLCDLPATPKGSGTSLFQHMLDLRAGKSLEDNPWLHEDVVTTETKSVVKEGIENHVYPTDMSTLPEKSLNDPPE

SEQ ID NO: 28 - protein, 786 aa, synthetic construct
  source 1..786: note = fusion protein gEgI(gE-A186V, L536I)
RITNPVRASVLRYDDFHIDEDKLDTNSVYEPYYHSDHAESSWVNRGESSRKAYDHNSPYIWPRNDYDGFLENAHEHHGVYNQGRGIDSGERLMQPTQMSAQEDLGDDTGIHVIPTLNGDDRHKIVNVDQRQYGDVFKGDLNPKPQGQRLIEVSVEENHPFTLRVPIQRIYGVRYTETWSFLPSLTCTGDAAPAIQHICLKHTTCFQDVVVDVDCAENTKEDQLAEISYRFQGKKEADQPWIVVNTSTLFDELELDPPEIEPGVLKVLRTEKQYLGVYIWNMRGSDGTSTYATFLVTWKGDEKTRNPTPAVTPQPRGAEFHMWNYHSHVFSVGDTFSLAMHLQYKIHEAPFDLLLEWLYVPIDPTCQPMRLYSTCLYHPNAPQCLSHMNSGCTFTSPHLAQRVASTVYQNCEHADNYTAYCLGISHMEPSFGLILHDGGTTLKFVDTPESLSGLYVFVVYFNGHVEAVAYTVVSTVDHFVNAIEERGFPPTAGQPPATTKPKEITPVNPGTSPLIRGGGGSGGGGSGGGGSGGGGSLIFKGDHVSLQVNSSLTSILIPMQNDNYTEIKGQLVFIGEQLPTGTNYSGTLELLYADTVAFCFRSVQVIRYDGCPRIRTSAFISCRYKHSWHYGNSTDRISTEPDAGVMLKITKPGINDAGVYVLLVRLDHSRSTDGFILGVNVYTAGSHHNIHGVIYTSPSLQNGYSTRALFQQARLCDLPATPKGSGTSLFQHMLDLRAGKSLEDNPWLHEDVVTTETKSVVKEGIENHVYPTDMSTLPEKSLNDPPE

SEQ ID NO: 29 - protein, 786 aa, synthetic construct
  source 1..786: note = fusion protein gEgI(gE-T512M, L536I)
RITNPVRASVLRYDDFHIDEDKLDTNSVYEPYYHSDHAESSWVNRGESSRKAYDHNSPYIWPRNDYDGFLENAHEHHGVYNQGRGIDSGERLMQPTQMSAQEDLGDDTGIHVIPTLNGDDRHKIVNVDQRQYGDVFKGDLNPKPQGQRLIEVSVEENHPFTLRAPIQRIYGVRYTETWSFLPSLTCTGDAAPAIQHICLKHTTCFQDVVVDVDCAENTKEDQLAEISYRFQGKKEADQPWIVVNTSTLFDELELDPPEIEPGVLKVLRTEKQYLGVYIWNMRGSDGTSTYATFLVTWKGDEKTRNPTPAVTPQPRGAEFHMWNYHSHVFSVGDTFSLAMHLQYKIHEAPFDLLLEWLYVPIDPTCQPMRLYSTCLYHPNAPQCLSHMNSGCTFTSPHLAQRVASTVYQNCEHADNYTAYCLGISHMEPSFGLILHDGGTTLKFVDTPESLSGLYVFVVYFNGHVEAVAYTVVSTVDHFVNAIEERGFPPMAGQPPATTKPKEITPVNPGTSPLIRGGGGSGGGGSGGGGSGGGGSLIFKGDHVSLQVNSSLTSILIPMQNDNYTEIKGQLVFIGEQLPTGTNYSGTLELLYADTVAFCFRSVQVIRYDGCPRIRTSAFISCRYKHSWHYGNSTDRISTEPDAGVMLKITKPGINDAGVYVLLVRLDHSRSTDGFILGVNVYTAGSHHNIHGVIYTSPSLQNGYSTRALFQQARLCDLPATPKGSGTSLFQHMLDLRAGKSLEDNPWLHEDVVTTETKSVVKEGIENHVYPTDMSTLPEKSLNDPPE

SEQ ID NO: 30 - protein, 786 aa, synthetic construct
  source 1..786: note = fusion protein gEgI(gI-T211P)
RITNPVRASVLRYDDFHIDEDKLDTNSVYEPYYHSDHAESSWVNRGESSRKAYDHNSPYIWPRNDYDGFLENAHEHHGVYNQGRGIDSGERLMQPTQMSAQEDLGDDTGIHVIPTLNGDDRHKIVNVDQRQYGDVFKGDLNPKPQGQRLIEVSVEENHPFTLRAPIQRIYGVRYTETWSFLPSLTCTGDAAPAIQHICLKHTTCFQDVVVDVDCAENTKEDQLAEISYRFQGKKEADQPWIVVNTSTLFDELELDPPEIEPGVLKVLRTEKQYLGVYIWNMRGSDGTSTYATFLVTWKGDEKTRNPTPAVTPQPRGAEFHMWNYHSHVFSVGDTFSLAMHLQYKIHEAPFDLLLEWLYVPIDPTCQPMRLYSTCLYHPNAPQCLSHMNSGCTFTSPHLAQRVASTVYQNCEHADNYTAYCLGISHMEPSFGLILHDGGTTLKFVDTPESLSGLYVFVVYFNGHVEAVAYTVVSTVDHFVNAIEERGFPPTAGQPPATTKPKEITPVNPGTSPLLRGGGGSGGGGSGGGGSGGGGSLIFKGDHVSLQVNSSLTSILIPMQNDNYTEIKGQLVFIGEQLPTGTNYSGTLELLYADTVAFCFRSVQVIRYDGCPRIRTSAFISCRYKHSWHYGNSTDRISTEPDAGVMLKITKPGINDAGVYVLLVRLDHSRSTDGFILGVNVYTAGSHHNIHGVIYTSPSLQNGYSTRALFQQARLCDLPATPKGSGPSLFQHMLDLRAGKSLEDNPWLHEDVVTTETKSVVKEGIENHVYPTDMSTLPEKSLNDPPE

SEQ ID NO: 31 - protein, 786 aa, synthetic construct
  source 1..786: note = fusion protein gEgI(gI-K246Q)
RITNPVRASVLRYDDFHIDEDKLDTNSVYEPYYHSDHAESSWVNRGESSRKAYDHNSPYIWPRNDYDGFLENAHEHHGVYNQGRGIDSGERLMQPTQMSAQEDLGDDTGIHVIPTLNGDDRHKIVNVDQRQYGDVFKGDLNPKPQGQRLIEVSVEENHPFTLRAPIQRIYGVRYTETWSFLPSLTCTGDAAPAIQHICLKHTTCFQDVVVDVDCAENTKEDQLAEISYRFQGKKEADQPWIVVNTSTLFDELELDPPEIEPGVLKVLRTEKQYLGVYIWNMRGSDGTSTYATFLVTWKGDEKTRNPTPAVTPQPRGAEFHMWNYHSHVFSVGDTFSLAMHLQYKIHEAPFDLLLEWLYVPIDPTCQPMRLYSTCLYHPNAPQCLSHMNSGCTFTSPHLAQRVASTVYQNCEHADNYTAYCLGISHMEPSFGLILHDGGTTLKFVDTPESLSGLYVFVVYFNGHVEAVAYTVVSTVDHFVNAIEERGFPPTAGQPPATTKPKEITPVNPGTSPLLRGGGGSGGGGSGGGGSGGGGSLIFKGDHVSLQVNSSLTSILIPMQNDNYTEIKGQLVFIGEQLPTGTNYSGTLELLYADTVAFCFRSVQVIRYDGCPRIRTSAFISCRYKHSWHYGNSTDRISTEPDAGVMLKITKPGINDAGVYVLLVRLDHSRSTDGFILGVNVYTAGSHHNIHGVIYTSPSLQNGYSTRALFQQARLCDLPATPKGSGTSLFQHMLDLRAGKSLEDNPWLHEDVVTTETKSVVQEGIENHVYPTDMSTLPEKSLNDPPE

SEQ ID NO: 32 - protein, 786 aa, synthetic construct
  source 1..786: note = fusion protein gEgI(gI-N267S)
RITNPVRASVLRYDDFHIDEDKLDTNSVYEPYYHSDHAESSWVNRGESSRKAYDHNSPYIWPRNDYDGFLENAHEHHGVYNQGRGIDSGERLMQPTQMSAQEDLGDDTGIHVIPTLNGDDRHKIVNVDQRQYGDVFKGDLNPKPQGQRLIEVSVEENHPFTLRAPIQRIYGVRYTETWSFLPSLTCTGDAAPAIQHICLKHTTCFQDVVVDVDCAENTKEDQLAEISYRFQGKKEADQPWIVVNTSTLFDELELDPPEIEPGVLKVLRTEKQYLGVYIWNMRGSDGTSTYATFLVTWKGDEKTRNPTPAVTPQPRGAEFHMWNYHSHVFSVGDTFSLAMHLQYKIHEAPFDLLLEWLYVPIDPTCQPMRLYSTCLYHPNAPQCLSHMNSGCTFTSPHLAQRVASTVYQNCEHADNYTAYCLGISHMEPSFGLILHDGGTTLKFVDTPESLSGLYVFVVYFNGHVEAVAYTVVSTVDHFVNAIEERGFPPTAGQPPATTKPKEITPVNPGTSPLLRGGGGSGGGGSGGGGSGGGGSLIFKGDHVSLQVNSSLTSILIPMQNDNYTEIKGQLVFIGEQLPTGTNYSGTLELLYADTVAFCFRSVQVIRYDGCPRIRTSAFISCRYKHSWHYGNSTDRISTEPDAGVMLKITKPGINDAGVYVLLVRLDHSRSTDGFILGVNVYTAGSHHNIHGVIYTSPSLQNGYSTRALFQQARLCDLPATPKGSGTSLFQHMLDLRAGKSLEDNPWLHEDVVTTETKSVVKEGIENHVYPTDMSTLPEKSLSDPPE

SEQ ID NO: 33 - protein, 515 aa, synthetic construct
  source 1..515: note = gE(aa. 23-537,I40T)
RITNPVRASVLRYDDFHTDEDKLDTNSVYEPYYHSDHAESSWVNRGESSRKAYDHNSPYIWPRNDYDGFLENAHEHHGVYNQGRGIDSGERLMQPTQMSAQEDLGDDTGIHVIPTLNGDDRHKIVNVDQRQYGDVFKGDLNPKPQGQRLIEVSVEENHPFTLRAPIQRIYGVRYTETWSFLPSLTCTGDAAPAIQHICLKHTTCFQDVVVDVDCAENTKEDQLAEISYRFQGKKEADQPWIVVNTSTLFDELELDPPEIEPGVLKVLRTEKQYLGVYIWNMRGSDGTSTYATFLVTWKGDEKTRNPTPAVTPQPRGAEFHMWNYHSHVFSVGDTFSLAMHLQYKIHEAPFDLLLEWLYVPIDPTCQPMRLYSTCLYHPNAPQCLSHMNSGCTFTSPHLAQRVASTVYQNCEHADNYTAYCLGISHMEPSFGLILHDGGTTLKFVDTPESLSGLYVFVVYFNGHVEAVAYTVVSTVDHFVNAIEERGFPPTAGQPPATTKPKEITPVNPGTSPLLR

SEQ ID NO: 34 - protein, 515 aa, synthetic construct
  source 1..515: note = gE(aa. 23-537, E124D)
RITNPVRASVLRYDDFHIDEDKLDTNSVYEPYYHSDHAESSWVNRGESSRKAYDHNSPYIWPRNDYDGFLENAHEHHGVYNQGRGIDSGERLMQPTQMSAQDDLGDDTGIHVIPTLNGDDRHKIVNVDQRQYGDVFKGDLNPKPQGQRLIEVSVEENHPFTLRAPIQRIYGVRYTETWSFLPSLTCTGDAAPAIQHICLKHTTCFQDVVVDVDCAENTKEDQLAEISYRFQGKKEADQPWIVVNTSTLFDELELDPPEIEPGVLKVLRTEKQYLGVYIWNMRGSDGTSTYATFLVTWKGDEKTRNPTPAVTPQPRGAEFHMWNYHSHVFSVGDTFSLAMHLQYKIHEAPFDLLLEWLYVPIDPTCQPMRLYSTCLYHPNAPQCLSHMNSGCTFTSPHLAQRVASTVYQNCEHADNYTAYCLGISHMEPSFGLILHDGGTTLKFVDTPESLSGLYVFVVYFNGHVEAVAYTVVSTVDHFVNAIEERGFPPTAGQPPATTKPKEITPVNPGTSPLLR

SEQ ID NO: 35 - protein, 515 aa, synthetic construct
  source 1..515: note = gE(aa. 23-537,L162R)
RITNPVRASVLRYDDFHIDEDKLDTNSVYEPYYHSDHAESSWVNRGESSRKAYDHNSPYIWPRNDYDGFLENAHEHHGVYNQGRGIDSGERLMQPTQMSAQEDLGDDTGIHVIPTLNGDDRHKIVNVDQRQYGDVFKGDRNPKPQGQRLIEVSVEENHPFTLRAPIQRIYGVRYTETWSFLPSLTCTGDAAPAIQHICLKHTTCFQDVVVDVDCAENTKEDQLAEISYRFQGKKEADQPWIVVNTSTLFDELELDPPEIEPGVLKVLRTEKQYLGVYIWNMRGSDGTSTYATFLVTWKGDEKTRNPTPAVTPQPRGAEFHMWNYHSHVFSVGDTFSLAMHLQYKIHEAPFDLLLEWLYVPIDPTCQPMRLYSTCLYHPNAPQCLSHMNSGCTFTSPHLAQRVASTVYQNCEHADNYTAYCLGISHMEPSFGLILHDGGTTLKFVDTPESLSGLYVFVVYFNGHVEAVAYTVVSTVDHFVNAIEERGFPPTAGQPPATTKPKEITPVNPGTSPLLR

SEQ ID NO: 36 - protein, 515 aa, synthetic construct
  source 1..515: note = gE(aa. 23-537, W319R)
RITNPVRASVLRYDDFHIDEDKLDTNSVYEPYYHSDHAESSWVNRGESSRKAYDHNSPYIWPRNDYDGFLENAHEHHGVYNQGRGIDSGERLMQPTQMSAQEDLGDDTGIHVIPTLNGDDRHKIVNVDQRQYGDVFKGDLNPKPQGQRLIEVSVEENHPFTLRAPIQRIYGVRYTETWSFLPSLTCTGDAAPAIQHICLKHTTCFQDVVVDVDCAENTKEDQLAEISYRFQGKKEADQPWIVVNTSTLFDELELDPPEIEPGVLKVLRTEKQYLGVYIWNMRGSDGTSTYATFLVTRKGDEKTRNPTPAVTPQPRGAEFHMWNYHSHVFSVGDTFSLAMHLQYKIHEAPFDLLLEWLYVPIDPTCQPMRLYSTCLYHPNAPQCLSHMNSGCTFTSPHLAQRVASTVYQNCEHADNYTAYCLGISHMEPSFGLILHDGGTTLKFVDTPESLSGLYVFVVYFNGHVEAVAYTVVSTVDHFVNAIEERGFPPTAGQPPATTKPKEITPVNPGTSPLLR

SEQ ID NO: 37 - protein, 515 aa, synthetic construct
  source 1..515: note = gE(aa. 23-537, L359S)
RITNPVRASVLRYDDFHIDEDKLDTNSVYEPYYHSDHAESSWVNRGESSRKAYDHNSPYIWPRNDYDGFLENAHEHHGVYNQGRGIDSGERLMQPTQMSAQEDLGDDTGIHVIPTLNGDDRHKIVNVDQRQYGDVFKGDLNPKPQGQRLIEVSVEENHPFTLRAPIQRIYGVRYTETWSFLPSLTCTGDAAPAIQHICLKHTTCFQDVVVDVDCAENTKEDQLAEISYRFQGKKEADQPWIVVNTSTLFDELELDPPEIEPGVLKVLRTEKQYLGVYIWNMRGSDGTSTYATFLVTWKGDEKTRNPTPAVTPQPRGAEFHMWNYHSHVFSVGDTFSSAMHLQYKIHEAPFDLLLEWLYVPIDPTCQPMRLYSTCLYHPNAPQCLSHMNSGCTFTSPHLAQRVASTVYQNCEHADNYTAYCLGISHMEPSFGLILHDGGTTLKFVDTPESLSGLYVFVVYFNGHVEAVAYTVVSTVDHFVNAIEERGFPPTAGQPPATTKPKEITPVNPGTSPLLR

SEQ ID NO: 38 - protein, 515 aa, synthetic construct
  source 1..515: note = gE(aa. 23-537, Q404K)
RITNPVRASVLRYDDFHIDEDKLDTNSVYEPYYHSDHAESSWVNRGESSRKAYDHNSPYIWPRNDYDGFLENAHEHHGVYNQGRGIDSGERLMQPTQMSAQEDLGDDTGIHVIPTLNGDDRHKIVNVDQRQYGDVFKGDLNPKPQGQRLIEVSVEENHPFTLRAPIQRIYGVRYTETWSFLPSLTCTGDAAPAIQHICLKHTTCFQDVVVDVDCAENTKEDQLAEISYRFQGKKEADQPWIVVNTSTLFDELELDPPEIEPGVLKVLRTEKQYLGVYIWNMRGSDGTSTYATFLVTWKGDEKTRNPTPAVTPQPRGAEFHMWNYHSHVFSVGDTFSLAMHLQYKIHEAPFDLLLEWLYVPIDPTCQPMRLYSTCLYHPNAPKCLSHMNSGCTFTSPHLAQRVASTVYQNCEHADNYTAYCLGISHMEPSFGLILHDGGTTLKFVDTPESLSGLYVFVVYFNGHVEAVAYTVVSTVDHFVNAIEERGFPPTAGQPPATTKPKEITPVNPGTSPLLR

SEQ ID NO: 39 - protein, 515 aa, synthetic construct
  source 1..515: note = gE(aa. 23-537, L536I)
RITNPVRASVLRYDDFHIDEDKLDTNSVYEPYYHSDHAESSWVNRGESSRKAYDHNSPYIWPRNDYDGFLENAHEHHGVYNQGRGIDSGERLMQPTQMSAQEDLGDDTGIHVIPTLNGDDRHKIVNVDQRQYGDVFKGDLNPKPQGQRLIEVSVEENHPFTLRAPIQRIYGVRYTETWSFLPSLTCTGDAAPAIQHICLKHTTCFQDVVVDVDCAENTKEDQLAEISYRFQGKKEADQPWIVVNTSTLFDELELDPPEIEPGVLKVLRTEKQYLGVYIWNMRGSDGTSTYATFLVTWKGDEKTRNPTPAVTPQPRGAEFHMWNYHSHVFSVGDTFSLAMHLQYKIHEAPFDLLLEWLYVPIDPTCQPMRLYSTCLYHPNAPQCLSHMNSGCTFTSPHLAQRVASTVYQNCEHADNYTAYCLGISHMEPSFGLILHDGGTTLKFVDTPESLSGLYVFVVYFNGHVEAVAYTVVSTVDHFVNAIEERGFPPTAGQPPATTKPKEITPVNPGTSPLIR

SEQ ID NO: 40 - protein, 515 aa, synthetic construct
  source 1..515: note = gE(aa. 23-537, I40T&D150N)
RITNPVRASVLRYDDFHTDEDKLDTNSVYEPYYHSDHAESSWVNRGESSRKAYDHNSPYIWPRNDYDGFLENAHEHHGVYNQGRGIDSGERLMQPTQMSAQEDLGDDTGIHVIPTLNGDDRHKIVNVNQRQYGDVFKGDLNPKPQGQRLIEVSVEENHPFTLRAPIQRIYGVRYTETWSFLPSLTCTGDAAPAIQHICLKHTTCFQDVVVDVDCAENTKEDQLAEISYRFQGKKEADQPWIVVNTSTLFDELELDPPEIEPGVLKVLRTEKQYLGVYIWNMRGSDGTSTYATFLVTWKGDEKTRNPTPAVTPQPRGAEFHMWNYHSHVFSVGDTFSLAMHLQYKIHEAPFDLLLEWLYVPIDPTCQPMRLYSTCLYHPNAPQCLSHMNSGCTFTSPHLAQRVASTVYQNCEHADNYTAYCLGISHMEPSFGLILHDGGTTLKFVDTPESLSGLYVFVVYFNGHVEAVAYTVVSTVDHFVNAIEERGFPPTAGQPPATTKPKEITPVNPGTSPLLR

SEQ ID NO: 41 - protein, 515 aa, synthetic construct
  source 1..515: note = gE(aa. 23-537, A186V&L536I)
RITNPVRASVLRYDDFHIDEDKLDTNSVYEPYYHSDHAESSWVNRGESSRKAYDHNSPYIWPRNDYDGFLENAHEHHGVYNQGRGIDSGERLMQPTQMSAQEDLGDDTGIHVIPTLNGDDRHKIVNVDQRQYGDVFKGDLNPKPQGQRLIEVSVEENHPFTLRVPIQRIYGVRYTETWSFLPSLTCTGDAAPAIQHICLKHTTCFQDVVVDVDCAENTKEDQLAEISYRFQGKKEADQPWIVVNTSTLFDELELDPPEIEPGVLKVLRTEKQYLGVYIWNMRGSDGTSTYATFLVTWKGDEKTRNPTPAVTPQPRGAEFHMWNYHSHVFSVGDTFSLAMHLQYKIHEAPFDLLLEWLYVPIDPTCQPMRLYSTCLYHPNAPQCLSHMNSGCTFTSPHLAQRVASTVYQNCEHADNYTAYCLGISHMEPSFGLILHDGGTTLKFVDTPESLSGLYVFVVYFNGHVEAVAYTVVSTVDHFVNAIEERGFPPTAGQPPATTKPKEITPVNPGTSPLIR

SEQ ID NO: 42 - protein, 515 aa, synthetic construct
  source 1..515: note = gE(aa. 23-537, T512M&L536I)
RITNPVRASVLRYDDFHIDEDKLDTNSVYEPYYHSDHAESSWVNRGESSRKAYDHNSPYIWPRNDYDGFLENAHEHHGVYNQGRGIDSGERLMQPTQMSAQEDLGDDTGIHVIPTLNGDDRHKIVNVDQRQYGDVFKGDLNPKPQGQRLIEVSVEENHPFTLRAPIQRIYGVRYTETWSFLPSLTCTGDAAPAIQHICLKHTTCFQDVVVDVDCAENTKEDQLAEISYRFQGKKEADQPWIVVNTSTLFDELELDPPEIEPGVLKVLRTEKQYLGVYIWNMRGSDGTSTYATFLVTWKGDEKTRNPTPAVTPQPRGAEFHMWNYHSHVFSVGDTFSLAMHLQYKIHEAPFDLLLEWLYVPIDPTCQPMRLYSTCLYHPNAPQCLSHMNSGCTFTSPHLAQRVASTVYQNCEHADNYTAYCLGISHMEPSFGLILHDGGTTLKFVDTPESLSGLYVFVVYFNGHVEAVAYTVVSTVDHFVNAIEERGFPPMAGQPPATTKPKEITPVNPGTSPLIR

SEQ ID NO: 43 - protein, 251 aa, synthetic construct
  source 1..251: note = gI(aa. 21-271, T211P)
LIFKGDHVSLQVNSSLTSILIPMQNDNYTEIKGQLVFIGEQLPTGTNYSGTLELLYADTVAFCFRSVQVIRYDGCPRIRTSAFISCRYKHSWHYGNSTDRISTEPDAGVMLKITKPGINDAGVYVLLVRLDHSRSTDGFILGVNVYTAGSHHNIHGVIYTSPSLQNGYSTRALFQQARLCDLPATPKGSGPSLFQHMLDLRAGKSLEDNPWLHEDVVTTETKSVVKEGIENHVYPTDMSTLPEKSLNDPPE

SEQ ID NO: 44 - protein, 251 aa, synthetic construct
  source 1..251: note = gI (aa. 21-271, K246Q)
LIFKGDHVSLQVNSSLTSILIPMQNDNYTEIKGQLVFIGEQLPTGTNYSGTLELLYADTVAFCFRSVQVIRYDGCPRIRTSAFISCRYKHSWHYGNSTDRISTEPDAGVMLKITKPGINDAGVYVLLVRLDHSRSTDGFILGVNVYTAGSHHNIHGVIYTSPSLQNGYSTRALFQQARLCDLPATPKGSGTSLFQHMLDLRAGKSLEDNPWLHEDVVTTETKSVVQEGIENHVYPTDMSTLPEKSLNDPPE

SEQ ID NO: 45 - protein, 251 aa, synthetic construct
  source 1..251: note = gI(aa. 21-271, N267S)
LIFKGDHVSLQVNSSLTSILIPMQNDNYTEIKGQLVFIGEQLPTGTNYSGTLELLYADTVAFCFRSVQVIRYDGCPRIRTSAFISCRYKHSWHYGNSTDRISTEPDAGVMLKITKPGINDAGVYVLLVRLDHSRSTDGFILGVNVYTAGSHHNIHGVIYTSPSLQNGYSTRALFQQARLCDLPATPKGSGTSLFQHMLDLRAGKSLEDNPWLHEDVVTTETKSVVKEGIENHVYPTDMSTLPEKSLSDPPE

SEQ ID NO: 46 - protein, 623 aa, synthetic construct
  source 1..623: note = gE in full-length (Dumas strain)
MGTVNKPVVGVLMGFGIITGTLRITNPVRASVLRYDDFHTDEDKLDTNSVYEPYYHSDHAESSWVNRGESSRKAYDHNSPYIWPRNDYDGFLENAHEHHGVYNQGRGIDSGERLMQPTQMSAQEDLGDDTGIHVIPTLNGDDRHKIVNVDQRQYGDVFKGDLNPKPQGQRLIEVSVEENHPFTLRAPIQRIYGVRYTETWSFLPSLTCTGDAAPAIQHICLKHTTCFQDVVVDVDCAENTKEDQLAEISYRFQGKKEADQPWIVVNTSTLFDELELDPPEIEPGVLKVLRTEKQYLGVYIWNMRGSDGTSTYATFLVTWKGDEKTRNPTPAVTPQPRGAEFHMWNYHSHVFSVGDTFSLAMHLQYKIHEAPFDLLLEWLYVPIDPTCQPMRLYSTCLYHPNAPQCLSHMNSGCTFTSPHLAQRVASTVYQNCEHADNYTAYCLGISHMEPSFGLILHDGGTTLKFVDTPESLSGLYVFVVYFNGHVEAVAYTVVSTVDHFVNAIEERGFPPTAGQPPATTKPKEITPVNPGTSPLLRYAAWTGGLAAVVLLCLVIFLICTAKRMRVKAYRVDKSPYNQSMYYAGLPVDDFEDSESTDTEEEFGNAIGGSHGGSSYTVYIDKTR

SEQ ID NO: 47 - protein, 623 aa, synthetic construct
  source 1..623: note = gE in full-length (MSP strain)
MGTVNKPVVGVLMGFGIITGTLRITNPVRASVLRYDDFHTDEDKLDTNSVYEPYYHSDHAESSWVNRGESSRKAYDHNSPYIWPRNDYDGFLENAHEHHGVYNQGRGIDSGERLMQPTQMSAQEDLGDDTGIHVIPTLNGDDRHKIVNVNQRQYGDVFKGDLNPKPQGQRLIEVSVEENHPFTLRAPIQRIYGVRYTETWSFLPSLTCTGDAAPAIQHICLKHTTCFQDVVVDVDCAENTKEDQLAEISYRFQGKKEADQPWIVVNTSTLFDELELDPPEIEPGVLKVLRTEKQYLGVYIWNMRGSDGTSTYATFLVTWKGDEKTRNPTPAVTPQPRGAEFHMWNYHSHVFSVGDTFSLAMHLQYKIHEAPFDLLLEWLYVPIDPTCQPMRLYSTCLYHPNAPQCLSHMNSGCTFTSPHLAQRVASTVYQNCEHADNYTAYCLGISHMEPSFGLILHDGGTTLKFVDTPESLSGLYVFVVYFNGHVEAVAYTVVSTVDHFVNAIEERGFPPTAGQPPATTKPKEITPVNPGTSPLLRYAAWTGGLAAVVLLCLVIFLICTAKRMRVKAYRVDKSPYNQSMYYAGLPVDDFEDSESTDTEEEFGNAIGGSHGGSSYTVYIDKTR

SEQ ID NO: 48 - protein, 623 aa, synthetic construct
  source 1..623: note = gE in full-length (GenBank: AEW88980)
MGTVNKPVVGVLMGFGIITGTLRITNPVRASVLRYDDFHIDEDKLDTNSVYEPYYHSDHAESSWVNRGESSRKAYDHNSPYIWPRNDYDGFLENAHEHHGVYNQGRGIDSGERLMQPTQMSAQEDLGDDTGIHVIPTLNGDDRHKIVNVDQRQYGDVFKGDLNPKPQGQRLIEVSVEENHPFTLRAPIQRIYGVRYTETWSFLPSLTCTGDAAPAIQHICLKHTTCFQDVVVDVDCAENTKEDQLAEISYRFQGKKEADQPWIVVNTSTLFDELELDPPEIEPGVLKVLRTEKQYLGVYIWNMRGSDGTSTYATFLVTWKGDEKTRNPTPAVTPQPRGAEFHMWNYHSHVFSVGDTFSLAMHLQYKIHEAPFDLLLEWLYVPIDPTCQPMRLYSTCLYHPNAPQCLSHMNSGCTFTSPHLAQRVASTVYQNCEHADNYTAYCLGISHMEPSFGLILHDGGTTLKFVDTPESLSGLYVFVVYFNGHVEAVAYTVVSTVDHFVNAIEERGFPPMAGQPPATTKPKEITPVNPGTSPLIRYAAWTGGLAAVVLLCLVIFLICTAKRMRVKAYRVDKSPYNQSMYYAGLPVDDFEDSESTDTEEEFGNAIGGSHRGSSYTVYIDKSP

SEQ ID NO: 49 - protein, 623 aa, synthetic construct
  source 1..623: note = gE in full-length (GenBank: AEW89124)
MGTVNKPVVGVLMGFGIITGTLRITNPVRASVLRYDDFHIDEDKLDTNSVYEPYYHSDHAESSWVNRGESSRKAYDHNSPYIWPRNDYDGFLENAHEHHGVYNQGRGIDSGERLMQPTQMSAQEDLGDDTGIHVIPTLNGDDRHKIVNVDQRQYGDVFKGDLNPKPQGQRLIEVSVEENHPFTLRAPIQRIYGVRYTETWSFLPSLTCTGDAAPAIQHICLKHTTCFQDVVVDVDCAENTKEDQLAEISYRFQGKKEADQPWIVVNTSTLFDELELDPPEIEPGVLKVLRTEKQYLGVYIWNMRGSDGTSTYATFLVTWKGDEKTRNPTPAVTPQPRGAEFHMWNYHSHVFSVGDTFSLAMHLQYKIHEAPFDLLLEWLYVPIDPTCQPMRLYSTCLYHPNAPKCLSHMNSGCTFTSPHLAQRVASTVYQNCEHADNYTAYCLGISHMEPSFGLILHDGGTTLKFVDTPESLSGLYVFVVYFNGHVEAVAYTVVSTVDHFVNAIEERGFPPTAGQPPATTKPKEITPVNPGTSPLLRYAAWTGGLAAVVLLCLVIFLICTAKRMRVKAYRVDKSPYNQSMYYAGLPVDDFEDSESTDTEEEFGNAIGGSHGGSSYTVYIDKTR

SEQ ID NO: 50 - protein, 623 aa, synthetic construct
  source 1..623: note = gE in full-length (GenBank: QCA43570)
MGTVNKPVVGVLMGFGIITGTLRITNPVRASVLRYDDFHIDEDKLDTNSVYEPYYHSDHAESSWVNRGESSRKAYDHNSPYIWPRNDYDGFLENAHEHHGVYNQGRGIDSGERLMQPTQMSAQEDLGDDTGIHVIPTLNGDDRHKIVNVDQRQYGDVFKGDLNPKPQGQRLIEVSVEENHPFTLRAPIQRIYGVRYTETWSFLPSLTCTGDAAPAIQHICLKHTTCFQDVVVDVDCAENTKEDQLAEISYRFQGKKEADQPWIVVNTSTLFDELELDPPEIEPGVLKVLRTEKQYLGVYIWNMRGSDGTSTYATFLVTRKGDEKTRNPTPAVTPQPRGAEFHMWNYHSHVFSVGDTFSLAMHLQYKIHEAPFDLLLEWLYVPIDPTCQPMRLYSTCLYHPNAPQCLSHMNSGCTFTSPHLAQRVASTVYQNCEHADNYTAYCLGISHMEPSFGLILHDGGTTLKFVDTPESLSGLYVFVVYFNGHVEAVAYTVVSTVDHFVNAIEERGFPPTAGQPPATTKPKEITPVNPGTSPLLRYAAWTGGLAAVVLLCLVIFLICTAKRMRVKAYRVDKSPYNQSMYYAGLPVDDFEDSESTDTEEEFGNAIGGSHGGSSYTVYIDKTR

SEQ ID NO: 51 - protein, 623 aa, synthetic construct
  source 1..623: note = gE in full-length (GenBank: QCA45176)
MGTVNKPVVGVLMGFGIITGTLRITNPVRASVLRYDDFHIDEDKLDTNSVYEPYYHSDHAESSWVNRGESSRKAYDHNSPYIWPRNDYDGFLENAHEHHGVYNQGRGIDSGERLMQPTQMSAQDDLGDDTGIHVIPTLNGDDRHKIVNVDQRQYGDVFKGDLNPKPQGQRLIEVSVEENHPFTLRAPIQRIYGVRYTETWSFLPSLTCTGDAAPAIQHICLKHTTCFQDVVVDVDCAENTKEDQLAEISYRFQGKKEADQPWIVVNTSTLFDELELDPPEIEPGVLKVLRTEKQYLGVYIWNMRGSDGTSTYATFLVTWKGDEKTRNPTPAVTPQPRGAEFHMWNYHSHVFSVGDTFSLAMHLQYKIHEAPFDLLLEWLYVPIDPTCQPMRLYSTCLYHPNAPQCLSHMNSGCTFTSPHLAQRVASTVYQNCEHADNYTAYCLGISHMEPSFGLILHDGGTTLKFVDTPESLSGLYVFVVYFNGHVEAVAYTVVSTVDHFVNAIEERGFPPTAGQPPATTKPKEITPVNPGTSPLLRYAAWTGGLAAVVLLCLVIFLICTAKRMRVKAYRVDKSPYNQSMYYAGLPVDDFEDSESTDTEEEFGNAIGGSHGGSSYTVYIDKTR

SEQ ID NO: 52 - protein, 623 aa, synthetic construct
  source 1..623: note = gE in full-length (GenBank: QWE79571)
MGTVNKPVVGVLMGFGIITGTLRITNPVRASVLRYDDFHIDEDKLDTNSVYEPYYHSDHAESSWVNRGESSRKAYDHNSPYIWPRNDYDGFLENAHEHHGVYNQGRGIDSGERLMQPTQMSAQEDLGDDTGIHVIPTLNGDDRHKIVNVDQRQYGDVFKGDLNPKPQGQRLIEVSVEENHPFTLRAPIQRIYGVRYTETWSFLPSLTCTGDAAPAIQHICLKHTTCFQDVVVDVDCAENTKEDQLAEISYRFQGKKEADQPWIVVNTSTLFDELELDPPEIEPGVLKVLRTEKQYLGVYIWNMRGSDGTSTYATFLVTWKGDEKTRNPTPAVTPQPRGAEFHMWNYHSHVFSVGDTFSSAMHLQYKIHEAPFDLLLEWLYVPIDPTCQPMRLYSTCLYHPNAPQCLSHMNSGCTFTSPHLAQRVASTVYQNCEHADNYTAYCLGISHMEPSFGLILHDGGTTLKFVDTPESLSGLYVFVVYFNGHVEAVAYTVVSTVDHFVNAIEERGFPPTAGQPPATTKPKEITPVNPGTSPLLRYAAWTGGLAAVVLLCLVIFLICTAKRMRVKAYRVDKSPYNQSMYYAGLPVDDFEDSESTDTEEEFGNAIGGSHGGSSYTVYIDKTR

SEQ ID NO: 53 - protein, 623 aa, synthetic construct
  source 1..623: note = gE in full-length (GenBank: AEW89412)
MGTVNKPVVGVLMGFGIITGTLRITNPVRASVLRYDDFHIDEDKLDTNSVYEPYYHSDHAESSWVNRGESSRKAYDHNSPYIWPRNDYDGFLENAHEHHGVYNQGRGIDSGERLMQPTQMSAQEDLGDDTGIHVIPTLNGDDRHKIVNVDQRQYGDVFKGDRNPKPQGQRLIEVSVEENHPFTLRAPIQRIYGVRYTETWSFLPSLTCTGDAAPAIQHICLKHTTCFQDVVVDVDCAENTKEDQLAEISYRFQGKKEADQPWIVVNTSTLFDELELDPPEIEPGVLKVLRTEKQYLGVYIWNMRGSDGTSTYATFLVTWKGDEKTRNPTPAVTPQPRGAEFHMWNYHSHVFSVGDTFSLAMHLQYKIHEAPFDLLLEWLYVPIDPTCQPMRLYSTCLYHPNAPQCLSHMNSGCTFTSPHLAQRVASTVYQNCEHADNYTAYCLGISHMEPSFGLILHDGGTTLKFVDTPESLSGLYVFVVYFNGHVEAVAYTVVSTVDHFVNAIEERGFPPTAGQPPATTKPKEITPVNPGTSPLLRYAAWTGGLAAVVLLCLVIFLICTAKRMRVKAYRVDKSPYNQSMYYAGLPVDDFEDSESTDTEEEFGNAIGGSHGGSSYTVYIDKTR

SEQ ID NO: 54 - protein, 623 aa, synthetic construct
  source 1..623: note = gE in full-length (GenBank: ANS12941)
MGTVNKPVVGVLMGFGIITGTLRITNPVRASVLRYDDFHIDEDKLDTNSVYEPYYHSDHAESSWVNRGESSRKAYDHNSPYIWPRNDYDGFLENAHEHHGVYNQGRGIDSGERLMQPTQMSAQEDLGDDTGIHVIPTLNGDDRHKIVNVDQRQYGDVFKGDLNPKPQGQRLIEVSVEENHPFTLRVPIQRIYGVRYTETWSFLPSLTCTGDAAPAIQHICLKHTTCFQDVVVDVDCAENTKEDQLAEISYRFQGKKEADQPWIVVNTSTLFDELELDPPEIEPGVLKVLRTEKQYLGVYIWNMRGSDGTSTYATFLVTWKGDEKTRNPTPAVTPQPRGAEFHMWNYHSHVFSVGDTFSLAMHLQYKIHEAPFDLLLEWLYVPIDPTCQPMRLYSTCLYHPNAPQCLSHMNSGCTFTSPHLAQRVASTVYQNCEHADNYTAYCLGISHMEPSFGLILHDGGTTLKFVDTPESLSGLYVFVVYFNGHVEAVAYTVVSTVDHFVNAIEERGFPPTAGQPPATTKPKEITPVNPGTSPLIRYAAWTGGLAAVVLLCLVIFLICTAKRMRVKAYRVDKSPYNQSMYYAGLPVDDFEDSESTDTEEEFGNAIGGSHGGSSYTVYIDKTR

SEQ ID NO: 55 - protein, 623 aa, synthetic construct
  source 1..623: note = gE in full-length (GenBank: AQT34120)
MGTVNKPVVGVLMGFGIITGTLRITNPVRASVLRYDDFHIDEDKLDTNSVYEPYYHSDHAESSWVNRGESSRKAYDHNSPYIWPRNDYDGFLENAHEHHGVYNQGRGIDSGERLMQPTQMSAQEDLGDDTGIHVIPTLNGDDRHKIVNVDQRQYGDVFKGDLNPKPQGQRLIEVSVEENHPFTLRAPIQRIYGVRYTETWSFLPSLTCTGDAAPAIQHICLKHTTCFQDVVVDVDCAENTKEDQLAEISYRFQGKKEADQPWIVVNTSTLFDELELDPPEIEPGVLKVLRTEKQYLGVYIWNMRGSDGTSTYATFLVTWKGDEKTRNPTPAVTPQPRGAEFHMWNYHSHVFSVGDTFSLAMHLQYKIHEAPFDLLLEWLYVPIDPTCQPMRLYSTCLYHPNAPQCLSHMNSGCTFTSPHLAQRVASTVYQNCEHADNYTAYCLGISHMEPSFGLILHDGGTTLKFVDTPESLSGLYVFVVYFNGHVEAVAYTVVSTVDHFVNAIEERGFPPTAGQPPATTKPKEITPVNPGTSPLIRYAAWTGGLAAVVLLCLVIFLICTAKRMRVKAYRVDKSPYNQSMYYAGLPVDDFEDSESTDTEEEFGNAIGGSHGGSSYTVYIDKTR

SEQ ID NO: 56 - protein, 354 aa, synthetic construct
  source 1..354: note = gI in full-length (GenBank: AEW89051)
MFLIQCLISAVIFYIQVTNALIFKGDHVSLQVNSSLTSILIPMQNDNYTEIKGQLVFIGEQLPTGTNYSGTLELLYADTVAFCFRSVQVIRYDGCPRIRTSAFISCRYKHSWHYGNSTDRISTEPDAGVMLKITKPGINDAGVYVLLVRLDHSRSTDGFILGVNVYTAGSHHNIHGVIYTSPSLQNGYSTRALFQQARLCDLPATPKGSGTSLFQHMLDLRAGKSLEDNPWLHEDVVTTETKSVVQEGIENHVYPTDMSTLPEKSLNDPPENLLIIIPIVASVMILTAMVIVIVISVKRRRIKKHPIYRPNTKTRRGIQNATPESDVMLEAAIAQLATIREESPPHSVVNPFVK

SEQ ID NO: 57 - protein, 354 aa, synthetic construct
  source 1..354: note = gI in full-length (GenBank: AEW89483)
MFLIQCLISAVIFYIQVTNALIFKGDHVSLQVNSSLTSILIPMQNDNYTEIKGQLVFIGEQLPTGTNYSGTLELLYADTVAFCFRSVQVIRYDGCPRIRTSAFISCRYKHSWHYGNSTDRISTEPDAGVMLKITKPGINDAGVYVLLVRLDHSRSTDGFILGVNVYTAGSHHNIHGVIYTSPSLQNGYSTRALFQQARLCDLPATPKGSGPSLFQHMLDLRAGKSLEDNPWLHEDVVTTETKSVVKEGIENHVYPTDMSTLPEKSLNDPPENLLIIIPIVASVMILTAMVIVIVISVKRRRIKKHPIYRPNTKTRRGIQNATPESDVMLEAAIAQLATIREESPPHSVVNPFVK

SEQ ID NO: 58 - protein, 354 aa, synthetic construct
  source 1..354: note = gI in full-length (GenBank: AGY34059)
MFLIQCLISAVIFYIQVTNALIFKGDHVSLQVNSSLTSILIPMQNDNYTEIKGQLVFIGEQLPTGTNYSGTLELLYADTVAFCFRSVQVIRYDGCPRIRTSAFISCRYKHSWHYGNSTDRISTEPDAGVMLKITKPGINDAGVYVLLVRLDHSRSTDGFILGVNVYTAGSHHNIHGVIYTSPSLQNGYSTRALFQQARLCDLPATPKGSGTSLFQHMLDLRAGKSLEDNPWLHEDVVTTETKSVVKEGIENHVYPTDMSTLPEKSLSDPPENLLIIIPIVASVMILTAMVIVIVISVKRRRIKKHPIYRPNTKTRRGIQNATPESDVMLEAAIAQLATIREESPPHSVVNPFVK

SEQ ID NO: 59 - protein, 746 aa, synthetic construct
  source 1..746: note = fusion protein gE(43-517)gI
DKLDTNSVYEPYYHSDHAESSWVNRGESSRKAYDHNSPYIWPRNDYDGFLENAHEHHGVYNQGRGIDSGERLMQPTQMSAQEDLGDDTGIHVIPTLNGDDRHKIVNVDQRQYGDVFKGDLNPKPQGQRLIEVSVEENHPFTLRAPIQRIYGVRYTETWSFLPSLTCTGDAAPAIQHICLKHTTCFQDVVVDVDCAENTKEDQLAEISYRFQGKKEADQPWIVVNTSTLFDELELDPPEIEPGVLKVLRTEKQYLGVYIWNMRGSDGTSTYATFLVTWKGDEKTRNPTPAVTPQPRGAEFHMWNYHSHVFSVGDTFSLAMHLQYKIHEAPFDLLLEWLYVPIDPTCQPMRLYSTCLYHPNAPQCLSHMNSGCTFTSPHLAQRVASTVYQNCEHADNYTAYCLGISHMEPSFGLILHDGGTTLKFVDTPESLSGLYVFVVYFNGHVEAVAYTVVSTVDHFVNAIEERGFPPTAGQPPGGGGSGGGGSGGGGSGGGGSLIFKGDHVSLQVNSSLTSILIPMQNDNYTEIKGQLVFIGEQLPTGTNYSGTLELLYADTVAFCFRSVQVIRYDGCPRIRTSAFISCRYKHSWHYGNSTDRISTEPDAGVMLKITKPGINDAGVYVLLVRLDHSRSTDGFILGVNVYTAGSHHNIHGVIYTSPSLQNGYSTRALFQQARLCDLPATPKGSGTSLFQHMLDLRAGKSLEDNPWLHEDVVTTETKSVVKEGIENHVYPTDMSTLPEKSLNDPPE

SEQ ID NO: 60 - protein, 706 aa, synthetic construct
  source 1..706: note = fusion protein gE(63-497)gI
SWVNRGESSRKAYDHNSPYIWPRNDYDGFLENAHEHHGVYNQGRGIDSGERLMQPTQMSAQEDLGDDTGIHVIPTLNGDDRHKIVNVDQRQYGDVFKGDLNPKPQGQRLIEVSVEENHPFTLRAPIQRIYGVRYTETWSFLPSLTCTGDAAPAIQHICLKHTTCFQDVVVDVDCAENTKEDQLAEISYRFQGKKEADQPWIVVNTSTLFDELELDPPEIEPGVLKVLRTEKQYLGVYIWNMRGSDGTSTYATFLVTWKGDEKTRNPTPAVTPQPRGAEFHMWNYHSHVFSVGDTFSLAMHLQYKIHEAPFDLLLEWLYVPIDPTCQPMRLYSTCLYHPNAPQCLSHMNSGCTFTSPHLAQRVASTVYQNCEHADNYTAYCLGISHMEPSFGLILHDGGTTLKFVDTPESLSGLYVFVVYFNGHVEAVAYTVVSTVGGGGSGGGGSGGGGSGGGGSLIFKGDHVSLQVNSSLTSILIPMQNDNYTEIKGQLVFIGEQLPTGTNYSGTLELLYADTVAFCFRSVQVIRYDGCPRIRTSAFISCRYKHSWHYGNSTDRISTEPDAGVMLKITKPGINDAGVYVLLVRLDHSRSTDGFILGVNVYTAGSHHNIHGVIYTSPSLQNGYSTRALFQQARLCDLPATPKGSGTSLFQHMLDLRAGKSLEDNPWLHEDVVTTETKSVVKEGIENHVYPTDMSTLPEKSLNDPPE

SEQ ID NO: 61 - protein, 666 aa, synthetic construct
  source 1..666: note = fusion protein gE(83-477)gI
WPRNDYDGFLENAHEHHGVYNQGRGIDSGERLMQPTQMSAQEDLGDDTGIHVIPTLNGDDRHKIVNVDQRQYGDVFKGDLNPKPQGQRLIEVSVEENHPFTLRAPIQRIYGVRYTETWSFLPSLTCTGDAAPAIQHICLKHTTCFQDVVVDVDCAENTKEDQLAEISYRFQGKKEADQPWIVVNTSTLFDELELDPPEIEPGVLKVLRTEKQYLGVYIWNMRGSDGTSTYATFLVTWKGDEKTRNPTPAVTPQPRGAEFHMWNYHSHVFSVGDTFSLAMHLQYKIHEAPFDLLLEWLYVPIDPTCQPMRLYSTCLYHPNAPQCLSHMNSGCTFTSPHLAQRVASTVYQNCEHADNYTAYCLGISHMEPSFGLILHDGGTTLKFVDTPESLSGLYVGGGGSGGGGSGGGGSGGGGSLIFKGDHVSLQVNSSLTSILIPMQNDNYTEIKGQLVFIGEQLPTGTNYSGTLELLYADTVAFCFRSVQVIRYDGCPRIRTSAFISCRYKHSWHYGNSTDRISTEPDAGVMLKITKPGINDAGVYVLLVRLDHSRSTDGFILGVNVYTAGSHHNIHGVIYTSPSLQNGYSTRALFQQARLCDLPATPKGSGTSLFQHMLDLRAGKSLEDNPWLHEDVVTTETKSVVKEGIENHVYPTDMSTLPEKSLNDPPE

SEQ ID NO: 62 - protein, 626 aa, synthetic construct
  source 1..626: note = fusion protein gE(103-457)gI
NQGRGIDSGERLMQPTQMSAQEDLGDDTGIHVIPTLNGDDRHKIVNVDQRQYGDVFKGDLNPKPQGQRLIEVSVEENHPFTLRAPIQRIYGVRYTETWSFLPSLTCTGDAAPAIQHICLKHTTCFQDVVVDVDCAENTKEDQLAEISYRFQGKKEADQPWIVVNTSTLFDELELDPPEIEPGVLKVLRTEKQYLGVYIWNMRGSDGTSTYATFLVTWKGDEKTRNPTPAVTPQPRGAEFHMWNYHSHVFSVGDTFSLAMHLQYKIHEAPFDLLLEWLYVPIDPTCQPMRLYSTCLYHPNAPQCLSHMNSGCTFTSPHLAQRVASTVYQNCEHADNYTAYCLGISHMEPSFGLILHGGGGSGGGGSGGGGSGGGGSLIFKGDHVSLQVNSSLTSILIPMQNDNYTEIKGQLVFIGEQLPTGTNYSGTLELLYADTVAFCFRSVQVIRYDGCPRIRTSAFISCRYKHSWHYGNSTDRISTEPDAGVMLKITKPGINDAGVYVLLVRLDHSRSTDGFILGVNVYTAGSHHNIHGVIYTSPSLQNGYSTRALFQQARLCDLPATPKGSGTSLFQHMLDLRAGKSLEDNPWLHEDVVTTETKSVVKEGIENHVYPTDMSTLPEKSLNDPPE

SEQ ID NO: 63 - protein, 546 aa, synthetic construct
  source 1..546: note = fusion protein gE(143-417)gI
RHKIVNVDQRQYGDVFKGDLNPKPQGQRLIEVSVEENHPFTLRAPIQRIYGVRYTETWSFLPSLTCTGDAAPAIQHICLKHTTCFQDVVVDVDCAENTKEDQLAEISYRFQGKKEADQPWIVVNTSTLFDELELDPPEIEPGVLKVLRTEKQYLGVYIWNMRGSDGTSTYATFLVTWKGDEKTRNPTPAVTPQPRGAEFHMWNYHSHVFSVGDTFSLAMHLQYKIHEAPFDLLLEWLYVPIDPTCQPMRLYSTCLYHPNAPQCLSHMNSGCTFTSGGGGSGGGGSGGGGSGGGGSLIFKGDHVSLQVNSSLTSILIPMQNDNYTEIKGQLVFIGEQLPTGTNYSGTLELLYADTVAFCFRSVQVIRYDGCPRIRTSAFISCRYKHSWHYGNSTDRISTEPDAGVMLKITKPGINDAGVYVLLVRLDHSRSTDGFILGVNVYTAGSHHNIHGVIYTSPSLQNGYSTRALFQQARLCDLPATPKGSGTSLFQHMLDLRAGKSLEDNPWLHEDVVTTETKSVVKEGIENHVYPTDMSTLPEKSLNDPPE

SEQ ID NO: 64 - protein, 475 aa, synthetic construct
  source 1..475: note = gE(aa. 43-517)
DKLDTNSVYEPYYHSDHAESSWVNRGESSRKAYDHNSPYIWPRNDYDGFLENAHEHHGVYNQGRGIDSGERLMQPTQMSAQEDLGDDTGIHVIPTLNGDDRHKIVNVDQRQYGDVFKGDLNPKPQGQRLIEVSVEENHPFTLRAPIQRIYGVRYTETWSFLPSLTCTGDAAPAIQHICLKHTTCFQDVVVDVDCAENTKEDQLAEISYRFQGKKEADQPWIVVNTSTLFDELELDPPEIEPGVLKVLRTEKQYLGVYIWNMRGSDGTSTYATFLVTWKGDEKTRNPTPAVTPQPRGAEFHMWNYHSHVFSVGDTFSLAMHLQYKIHEAPFDLLLEWLYVPIDPTCQPMRLYSTCLYHPNAPQCLSHMNSGCTFTSPHLAQRVASTVYQNCEHADNYTAYCLGISHMEPSFGLILHDGGTTLKFVDTPESLSGLYVFVVYFNGHVEAVAYTVVSTVDHFVNAIEERGFPPTAGQPP

SEQ ID NO: 65 - protein, 435 aa, synthetic construct
  source 1..435: note = gE(aa. 63-497)
SWVNRGESSRKAYDHNSPYIWPRNDYDGFLENAHEHHGVYNQGRGIDSGERLMQPTQMSAQEDLGDDTGIHVIPTLNGDDRHKIVNVDQRQYGDVFKGDLNPKPQGQRLIEVSVEENHPFTLRAPIQRIYGVRYTETWSFLPSLTCTGDAAPAIQHICLKHTTCFQDVVVDVDCAENTKEDQLAEISYRFQGKKEADQPWIVVNTSTLFDELELDPPEIEPGVLKVLRTEKQYLGVYIWNMRGSDGTSTYATFLVTWKGDEKTRNPTPAVTPQPRGAEFHMWNYHSHVFSVGDTFSLAMHLQYKIHEAPFDLLLEWLYVPIDPTCQPMRLYSTCLYHPNAPQCLSHMNSGCTFTSPHLAQRVASTVYQNCEHADNYTAYCLGISHMEPSFGLILHDGGTTLKFVDTPESLSGLYVFVVYFNGHVEAVAYTVVSTV

SEQ ID NO: 66 - protein, 395 aa, synthetic construct
  source 1..395: note = gE(aa. 83-477)
WPRNDYDGFLENAHEHHGVYNQGRGIDSGERLMQPTQMSAQEDLGDDTGIHVIPTLNGDDRHKIVNVDQRQYGDVFKGDLNPKPQGQRLIEVSVEENHPFTLRAPIQRIYGVRYTETWSFLPSLTCTGDAAPAIQHICLKHTTCFQDVVVDVDCAENTKEDQLAEISYRFQGKKEADQPWIVVNTSTLFDELELDPPEIEPGVLKVLRTEKQYLGVYIWNMRGSDGTSTYATFLVTWKGDEKTRNPTPAVTPQPRGAEFHMWNYHSHVFSVGDTFSLAMHLQYKIHEAPFDLLLEWLYVPIDPTCQPMRLYSTCLYHPNAPQCLSHMNSGCTFTSPHLAQRVASTVYQNCEHADNYTAYCLGISHMEPSFGLILHDGGTTLKFVDTPESLSGLYV

SEQ ID NO: 67 - protein, 355 aa, synthetic construct
  source 1..355: note = gE(aa. 103-457)
NQGRGIDSGERLMQPTQMSAQEDLGDDTGIHVIPTLNGDDRHKIVNVDQRQYGDVFKGDLNPKPQGQRLIEVSVEENHPFTLRAPIQRIYGVRYTETWSFLPSLTCTGDAAPAIQHICLKHTTCFQDVVVDVDCAENTKEDQLAEISYRFQGKKEADQPWIVVNTSTLFDELELDPPEIEPGVLKVLRTEKQYLGVYIWNMRGSDGTSTYATFLVTWKGDEKTRNPTPAVTPQPRGAEFHMWNYHSHVFSVGDTFSLAMHLQYKIHEAPFDLLLEWLYVPIDPTCQPMRLYSTCLYHPNAPQCLSHMNSGCTFTSPHLAQRVASTVYQNCEHADNYTAYCLGISHMEPSFGLILH

SEQ ID NO: 68 - protein, 275 aa, synthetic construct
  source 1..275: note = gE(aa. 143-417)
RHKIVNVDQRQYGDVFKGDLNPKPQGQRLIEVSVEENHPFTLRAPIQRIYGVRYTETWSFLPSLTCTGDAAPAIQHICLKHTTCFQDVVVDVDCAENTKEDQLAEISYRFQGKKEADQPWIVVNTSTLFDELELDPPEIEPGVLKVLRTEKQYLGVYIWNMRGSDGTSTYATFLVTWKGDEKTRNPTPAVTPQPRGAEFHMWNYHSHVFSVGDTFSLAMHLQYKIHEAPFDLLLEWLYVPIDPTCQPMRLYSTCLYHPNAPQCLSHMNSGCTFTS

SEQ ID NO: 69 - protein, 507 aa, synthetic construct
  source 1..507: note = gE(aa. 31-537)
SVLRYDDFHIDEDKLDTNSVYEPYYHSDHAESSWVNRGESSRKAYDHNSPYIWPRNDYDGFLENAHEHHGVYNQGRGIDSGERLMQPTQMSAQEDLGDDTGIHVIPTLNGDDRHKIVNVDQRQYGDVFKGDLNPKPQGQRLIEVSVEENHPFTLRAPIQRIYGVRYTETWSFLPSLTCTGDAAPAIQHICLKHTTCFQDVVVDVDCAENTKEDQLAEISYRFQGKKEADQPWIVVNTSTLFDELELDPPEIEPGVLKVLRTEKQYLGVYIWNMRGSDGTSTYATFLVTWKGDEKTRNPTPAVTPQPRGAEFHMWNYHSHVFSVGDTFSLAMHLQYKIHEAPFDLLLEWLYVPIDPTCQPMRLYSTCLYHPNAPQCLSHMNSGCTFTSPHLAQRVASTVYQNCEHADNYTAYCLGISHMEPSFGLILHDGGTTLKFVDTPESLSGLYVFVVYFNGHVEAVAYTVVSTVDHFVNAIEERGFPPTAGQPPATTKPKEITPVNPGTSPLLR

SEQ ID NO: 70 - protein, 778 aa, synthetic construct
  source 1..778: note = fusion protein gE(31-537)gI
SVLRYDDFHIDEDKLDTNSVYEPYYHSDHAESSWVNRGESSRKAYDHNSPYIWPRNDYDGFLENAHEHHGVYNQGRGIDSGERLMQPTQMSAQEDLGDDTGIHVIPTLNGDDRHKIVNVDQRQYGDVFKGDLNPKPQGQRLIEVSVEENHPFTLRAPIQRIYGVRYTETWSFLPSLTCTGDAAPAIQHICLKHTTCFQDVVVDVDCAENTKEDQLAEISYRFQGKKEADQPWIVVNTSTLFDELELDPPEIEPGVLKVLRTEKQYLGVYIWNMRGSDGTSTYATFLVTWKGDEKTRNPTPAVTPQPRGAEFHMWNYHSHVFSVGDTFSLAMHLQYKIHEAPFDLLLEWLYVPIDPTCQPMRLYSTCLYHPNAPQCLSHMNSGCTFTSPHLAQRVASTVYQNCEHADNYTAYCLGISHMEPSFGLILHDGGTTLKFVDTPESLSGLYVFVVYFNGHVEAVAYTVVSTVDHFVNAIEERGFPPTAGQPPATTKPKEITPVNPGTSPLLRGGGGSGGGGSGGGGSGGGGSLIFKGDHVSLQVNSSLTSILIPMQNDNYTEIKGQLVFIGEQLPTGTNYSGTLELLYADTVAFCFRSVQVIRYDGCPRIRTSAFISCRYKHSWHYGNSTDRISTEPDAGVMLKITKPGINDAGVYVLLVRLDHSRSTDGFILGVNVYTAGSHHNIHGVIYTSPSLQNGYSTRALFQQARLCDLPATPKGSGTSLFQHMLDLRAGKSLEDNPWLHEDVVTTETKSVVKEGIENHVYPTDMSTLPEKSLNDPPE

SEQ ID NO: 71 - RNA, 2358 nt, synthetic construct
  source 1..2358: mol_type = other RNA; note = RNA sequence encoding the fusion protein
cgtataacgaatccggtcagagcatccgtcttgcgatacgatgattttcacatcgatgaagacaaactggatacaaactccgtatatgagccttactaccattcagatcatgcggagtcttcatgggtaaatcggggagagtcttcgcgaaaagcgtacgatcataactcaccttatatatggccacgtaatgattatgatggatttttagagaacgcacacgaacaccatggggtgtataatcagggccgtggtatcgatagcggggaacggttaatgcaacccacacaaatgtctgcacaggaggatcttggggacgatacgggcatccacgttatccctacgttaaacggcgatgacagacataaaattgtaaatgtggaccaacgtcaatacggtgacgtgtttaaaggagatcttaatccaaaaccccaaggccaaagactcattgaggtgtcagtggaagaaaatcacccgtttactttacgcgcaccgattcagcggatttatggagtccggtacaccgagacttggagctttttgccgtcattaacctgtacgggagacgcagcgcccgccatccagcatatatgtttaaaacatacaacatgctttcaagacgtggtggtggatgtggattgcgcggaaaatactaaagaggatcagttggccgaaatcagttaccgttttcaaggtaagaaggaagcggaccaaccgtggattgttgtaaacacgagcacactgtttgatgaactcgaattagacccccccgagattgaaccgggtgtcttgaaagtacttcggacagaaaaacaatacttgggtgtgtacatttggaacatgcgcggctccgatggtacgtctacctacgccacgtttttggtcacctggaaaggggatgaaaaaacaagaaaccctacgcccgcagtaactcctcaaccaagaggggctgagtttcatatgtggaattaccactcgcatgtattttcagttggtgatacgtttagcttggcaatgcatcttcagtataagatacatgaagcgccatttgatttgctgttagagtggttgtatgtccccatcgatcctacatgtcaaccaatgcggttatattctacgtgtttgtatcatcccaacgcaccccaatgcctctctcatatgaattccggttgtacatttacctcgccacatttagcccagcgtgttgcaagcacagtgtatcaaaattgtgaacatgcagataactacaccgcatattgtctgggaatatctcatatggagcctagctttggtctaatcttacacgacgggggcaccacgttaaagtttgtagatacacccgagagtttgtcgggattatacgtttttgtggtgtattttaacgggcatgttgaagccgtagcatacactgttgtatccacagtagatcattttgtaaacgcaattgaagagcgtggatttccgccaacggccggtcagccaccggcgactactaaacccaaggaaattacccccgtaaaccccggaacgtcaccacttctacgaggagggggagggtcaggagggggagggtcaggagggggagggtcaggagggggagggtcattgatcttcaagggcgaccacgtgagcttgcaagttaacagcagtctcacgtctatccttattcccatgcaaaatgataattatacagagataaaaggacagcttgtctttattggagagcaactacctaccgggacaaactatagcggaacactggaactgttatacgcggatacggtggcgttttgtttccggtcagtacaagtaataagatacgacggatgtccccggattagaacgagcgcttttatttcgtgtaggtacaaacattcgtggcattatggtaactcaacggatcggatatcaacagagccggatgctggtgtaatgttgaaaattaccaaaccgggaataaatgatgctggtgtgtatgtacttcttgttcggttagaccatagcagatccaccgatggtttcattcttggtgtaaatgtatatacagcgggctcgcatcacaacattcacggggttatctacacttctccatctctacagaatggatattctacaagagccctttttcaacaagctcgtttgtgtgatttacccgcgacacccaaagggtccggtacctccctgtttcaacatatgcttgatcttcgtgccggtaaatcgttagaggataacccttggttacatgaggacgttgttacgacagaaactaagtccgttgttaaggaggggatagaaaatcacgtatatccaacggatatgtccacgttacccgaaaagtcccttaatgatcctccagaa

SEQ ID NO: 72 - skipped